European Patent Application EP 4 119 156 A1, published January 18, 2023. Title: PHARMACEUTICAL COMPOSITION FOR TREATMENT AND/OR PREVENTION OF CANCER. Applicant: TORAY Industries, Inc. The sequence listing filed with the application follows.

SEQUENCE LISTING (309 sequences)

SEQ ID NO: 1 - DNA, 5562 bp, Homo sapiens
  CDS (190)..(2319)
cagagggctgctggctggctaagtccctcccgctcccggctctcgcctcactaggagcggctctcggtgcagcgggacagggcgaagcggcctgcgcccacggagcgcgcgacactgcccggaagggaccgccacccttgccccctcagctgcccactcgtgatttccagcggcctccgcgcgcgcacgatgccctcggccaccagccacagcgggagcggcagcaagtcgtccggaccgccaccgccgtcgggttcctccgggagtgaggcggccgcgggagccggggccgccgcgccggcttctcagcaccccgcaaccggcaccggcgctgtccagaccgaggccatgaagcagattctcggggtgatcgacaagaaacttcggaacctggagaagaaaaagggtaagcttgatgattaccaggaacgaatgaacaaaggggaaaggcttaatcaagatcagctggatgccgtttctaagtaccaggaagtcacaaataatttggagtttgcaaaagaattacagaggagtttcatggcactaagtcaagatattcagaaaacaataaagaagacagcacgtcgggagcagcttatgagagaagaagctgaacagaaacgtttaaaaactgtacttgagctacagtatgttttggacaaattgggagatgatgaagtgcggactgacctgaaacaaggtttgaatggagtgccaatattgtccgaagaggagttgtcattgttggatgaattctataagctagtagaccctgaacgggacatgagcttgaggttgaatgaacagtatgaacatgcctccattcacctgtgggacctgctggaagggaaggaaaaacctgtatgtggaaccacctataaagttctaaaggaaattgttgagcgtgtttttcagtcaaactactttgacagcacccacaaccaccagaatgggctgtgtgaggaagaagaggcagcctcagcacctgcagttgaagaccaggtacctgaagctgaacctgagccagcagaagagtacactgagcaaagtgaagttgaatcaacagagtatgtaaatagacagttcatggcagaaacacagttcaccagtggtgaaaaggagcaggtagatgagtggacagttgaaacggttgaggtggtaaattcactccagcagcaacctcaggctgcatccccttcagtaccagagccccactctttgactccagtggctcaggcagatccccttgtgagaagacagcgagtacaagaccttatggcacaaatgcagggtccctataatttcatacaggattcaatgctggattttgaaaatcagacacttgatcctgccattgtatctgcacagcctatgaatccaacacaaaacatggacatgccccagctggtttgccctccagttcattctgaatctagacttgctcagcctaatcaagttcctgtacaaccagaagcgacacaggttcctttggtatcatccacaagtgaggggtacacagcatctcaacccttgtaccagccttctcatgctacagagcaacgaccacagaaggaaccaattgatcagattcaggcaacaatctctttaaatacagaccagactacagcatcatcatcccttcctgctgcgtctcagcctcaagtatttcaggctgggacaagcaaacctttacatagcagtggaatcaatgtaaatgcagctccattccaatccatgcaaacggtgttcaatatgaatgccccagttcctcctgttaatgaaccagaaactttaaaacagcaaaatcagtaccaggccagttataaccagagcttttctagtcagcctcaccaagtagaacaaacagagcttcagcaagaacagcttcaaacagtggttggcacttaccatggttccccagaccagtcccatcaagtgactggtaaccaccagcagcctcctcagcagaacactggatttccacgtagcaatcagccctattacaatagtcgtggtgtgtctcgtggaggctcccgtggtgctagaggcttgatgaatggataccggggccctgccaatggattcagaggaggatatgatggttaccgcccttcattctctaacactccaaacagtggttatacacagtctcagttcagtgctccccgggattactctggctatcaacgggatggatatcagcagaatttcaagcgaggctctgggcagagtggaccacggggagccccacgaggtcgtggagggcccccaagacccaacagagggatgccgcaaatgaacactcagcaagtgaattaatctgattcacaggattatgtttaatcgccaaaaacacactggccagtgtaccataatatgttaccagaagagttattatctatttgttctccctttcaggaaacttattgtaaagggactgttttcatcccataaagacaggactacaattgtcagctttctattacctggatatggaaggaaactatttttactctgcatgttctgtcctaagcgtcatcttgagccttgcacatgatactcagattcctcacccttgcttaggagtaaaacaatatactttacagggtgataataatctccatagttatttgaagtggcttgaaaaaggcaagattgacttttatgacattggataaaatctacaaatcagccctcgagttattcaatgataactgacaaactaaattatttccctagaaaggaagatgaaaggagtggagtgtggtttggcagaacaactgcatttcacagcttttccagttaaattggagcactgaacgttcagatgcataccaaattatgcatgggtcctaatcacacatataaggctggctaccagctttgacacagcactgttcatctggccaaacaactgtggttaaaaacacatgtaaaatgctttttaacagctgatactgtataagacaaagccaagatgcaaaattaggctttgattggcactttttgaaaaatatgcaacaaatatgggatgtaatccggatggccgcttctgtacttaatgtgaaatatttagatacctttttgaacacttaacagtttctttgagacaatgacttttgtaaggattggtactatctatcattccttatgacatgtacattgtctgtcactaatccttggattttgctgtattgtcacctaaattggtacaggtactgatgaaaatctctagtggataatcataacactctcggtcacatgtttttccttcagcttgaaagcttttttttaaaaggaaaagataccaaatgcctgctgctaccacccttttcaattgctatcttttgaaaggcaccagtatgtgttttagattgatttccctgtttcagggaaatcacggacagtagtttcagttctgatggtataagcaaaacaaataaaacgtttataaaagttgtatcttgaaacactggtgttcaacagctagcagcttatgtgattcaccccatgccacgttagtgtcacaaattttatggtttatctccagcaacatttctctagtacttgcacttattatcttttgtctaatttaaccttaactgaattctccgtttctcctggaggcatttatattcagtgataattccttcccttagatgcatagggagagtctctaaatttgatggaaatggacacttgagtagtgacttagccttatgtactctgttggaatttgtgctagcagtttgagcactagttctgtgtgcctaggaagttaatgctgcttattgtctcattctgacttcatggagaattaatcccacctttaagcaaaggctactaagttaatggtattttctgtgcagaaattaaattttattttcagcatttagcccaggaattcttccagtaggtgctcagctatttaaaaacaaaactattctcaaacattcatcattagacaactggagtttttgctggttttgtaacctaccaaaatggataggctgttgaacattccacattcaaaagttttgtagggtggtgggaaatgggggatcttcaatgtttattttaaaataaaataaaataagttcttgacttttctcatgtgtggttgtggtacatcatattggaagggttaacctgttactttggcaaatgagtatttttttgctagcacctccccttgcgtgctttaaatgacatctgcctgggatgtaccacaaccatatgttacctgtatcttaggggaatggataaaatatttgtggtttactgggtaatccctagatgatgtatgcttgcagtcctatataaaactaaatttgctatctgtgtagaaaataatttcatgacatttacaatcaggactgaagtaagttcttcacacagtgacctctgaatcagtttcagagaagggatgggggagaaaatgccttctaggttttgaacttctatgcattagtgcagatgttgtgaatgtgtaaaggtgttcatagtttgactgtttctatgtatgttttttcaaagaattgttcctttttttgaactataatttttctttttttggttattttaccatcacagtttaaatgtatatcttttatgtctctactcagaccatatttttaaaggggtgcctcattatggggcagagaacttttcaataagtctcattaagatctgaatcttggttctaagcattctgtataatatgtgattgcttgtcctagctgcagaaggccttttgtttggtcaaatgcatattttagcagagtttcaaggaaatgattgtcacacatgtcactgtagcctcttggtgtagcaagctcacatacaaaatacttttgtatatgcataatataaatcatctcatgtggatatgaaacttcttttttaaaacttaaaaaggtagaatgttattgattaccttgattagggcagttttatttccagatcctaataattcctaaaaaatatggaaaagttttttttcaatcattgtaccttgatattaaaacaaatatcctttaagtatttctaatcagttagcttctacagttcttttgtctccttttatatgcagctcttacgtgggagacttttccacttaaaggagacatagaatgtgtgcttattctcagaaggttcattaactgaggtgatgagttaacaactagttgagcagtcagcttcctaagtgttttaggacatttgttcattatattttccgtcatataactagaggaagtggaatgcagataagtgccgaattcaaacccttcattttatgtttaagctcctgaatctgcattccacttgggttgtttttaagcattctaaattttagttgattataagttagatttcacagaatcagtattgcccttgatcttgtcctttttatggagttaacggggaggaagacccctcaggaaaacgaaagtaaattgttaaggctcatcttcatacctttttccattttgaatcctacaaaaatactgcaaaagactagtgaatgtttaaaattacactagattaaataatatgaaagtc

SEQ ID NO: 2 - protein, 709 aa, Homo sapiens
MPSATSHSGSGSKSSGPPPPSGSSGSEAAAGAGAAAPASQHPATGTGAVQTEAMKQILGVIDKKLRNLEKKKGKLDDYQERMNKGERLNQDQLDAVSKYQEVTNNLEFAKELQRSFMALSQDIQKTIKKTARREQLMREEAEQKRLKTVLELQYVLDKLGDDEVRTDLKQGLNGVPILSEEELSLLDEFYKLVDPERDMSLRLNEQYEHASIHLWDLLEGKEKPVCGTTYKVLKEIVERVFQSNYFDSTHNHQNGLCEEEEAASAPAVEDQVPEAEPEPAEEYTEQSEVESTEYVNRQFMAETQFTSGEKEQVDEWTVETVEVVNSLQQQPQAASPSVPEPHSLTPVAQADPLVRRQRVQDLMAQMQGPYNFIQDSMLDFENQTLDPAIVSAQPMNPTQNMDMPQLVCPPVHSESRLAQPNQVPVQPEATQVPLVSSTSEGYTASQPLYQPSHATEQRPQKEPIDQIQATISLNTDQTTASSSLPAASQPQVFQAGTSKPLHSSGINVNAAPFQSMQTVFNMNAPVPPVNEPETLKQQNQYQASYNQSFSSQPHQVEQTELQQEQLQTVVGTYHGSPDQSHQVTGNHQQPPQQNTGFPRSNQPYYNSRGVSRGGSRGARGLMNGYRGPANGFRGGYDGYRPSFSNTPNSGYTQSQFSAPRDYSGYQRDGYQQNFKRGSGQSGPRGAPRGRGGPPRPNRGMPQMNTQQVN

SEQ ID NO: 3 - DNA, 3553 bp, Homo sapiens
  CDS (190)..(2274)
cagagggctgctggctggctaagtccctcccgctcccggctctcgcctcactaggagcggctctcggtgcagcgggacagggcgaagcggcctgcgcccacggagcgcgcgacactgcccggaagggaccgccacccttgccccctcagctgcccactcgtgatttccagcggcctccgcgcgcgcacgatgccctcggccaccagccacagcgggagcggcagcaagtcgtccggaccgccaccgccgtcgggttcctccgggagtgaggcggccgcgggagccggggccgccgcgccggcttctcagcaccccgcaaccggcaccggcgctgtccagaccgaggccatgaagcagattctcggggtgatcgacaagaaacttcggaacctggagaagaaaaagggtaagcttgatgattaccaggaacgaatgaacaaaggggaaaggcttaatcaagatcagctggatgccgtttctaagtaccaggaagtcacaaataatttggagtttgcaaaagaattacagaggagtttcatggcactaagtcaagatattcagaaaacaataaagaagacagcacgtcgggagcagcttatgagagaagaagctgaacagaaacgtttaaaaactgtacttgagctacagtatgttttggacaaattgggagatgatgaagtgcggactgacctgaaacaaggtttgaatggagtgccaatattgtccgaagaggagttgtcattgttggatgaattctataagctagtagaccctgaacgggacatgagcttgaggttgaatgaacagtatgaacatgcctccattcacctgtgggacctgctggaagggaaggaaaaacctgtatgtggaaccacctataaagttctaaaggaaattgttgagcgtgtttttcagtcaaactactttgacagcacccacaaccaccagaatgggctgtgtgaggaagaagaggcagcctcagcacctgcagttgaagaccaggtacctgaagctgaacctgagccagcagaagagtacactgagcaaagtgaagttgaatcaacagagtatgtaaatagacagttcatggcagaaacacagttcaccagtggtgaaaaggagcaggtagatgagtggacagttgaaacggttgaggtggtaaattcactccagcagcaacctcaggctgcatccccttcagtaccagagccccactctttgactccagtggctcaggcagatccccttgtgagaagacagcgagtacaagaccttatggcacaaatgcagggtccctataatttcatacaggattcaatgctggattttgaaaatcagacacttgatcctgccattgtatctgcacagcctatgaatccaacacaaaacatggacatgccccagctggtttgccctccagttcattctgaatctagacttgctcagcctaatcaagttcctgtacaaccagaagcgacacaggttcctttggtatcatccacaagtgaggggtacacagcatctcaacccttgtaccagccttctcatgctacagagcaacgaccacagaaggaaccaattgatcagattcaggcaacaatctctttaaatacagaccagactacagcatcatcatcccttcctgctgcgtctcagcctcaagtatttcaggctgggacaagcaaacctttacatagcagtggaatcaatgtaaatgcagctccattccaatccatgcaaacggtgttcaatatgaatgccccagttcctcctgttaatgaaccagaaactttaaaacagcaaaatcagtaccaggccagttataaccagagcttttctagtcagcctcaccaagtagaacaaacagagcttcagcaagaacagcttcaaacagtggttggcacttaccatggttccccagaccagtcccatcaagtgactggtaaccaccagcagcctcctcagcagaacactggatttccacgtagcaatcagccctattacaatagtcgtggtgtgtctcgtggaggctcccgtggtgctagaggcttgatgaatggataccggggccctgccaatggattcagaggaggatatgatggttaccgcccttcattctctaacactccaaacagtggttatacacagtctcagttcagtgctccccgggattactctggctatcaacgggatggatatcagcagaatttcaagcgaggctctgggcagagtggaccacggggagccccacgaggtaatattttgtggtggtgatcctagctcctaagtggagcttctgttctggccttggaagagctgttaatagtctgcatgttaggaatacatttatcctttccagacttgttgctagggattaaatgaaatgctctgtttctaaaacttaatcttggacccaaattttaatttttgaatgatttaattttccctgttactatataaactgtcttgaaaactagaacatattctcttctcagaaaaagtgtttttccaactgaaaattatttttcaggtcctaaaacctgctaaatgtttttaggaagtacttactgaaacatttttgtaagacatttttggaatgagattgaacatttatataaatttattattcctctttcatttttttgaaacatgcctattatattttagggccagacaccctttaatggccggataagccatagttaacatttagagaaccatttagaagtgatagaactaatggaatttgcaatgccttttggacctctattagtgatataaatatcaagttatttctgacttttaaacaaaactcccaaattcctaacttattgagctatacttaaaaaaaattacaggtttagagagttttttgtttttcttttactgttggaaaactacttcccattttggcaggaagttaacctatttaacaattagagctagcatttcatgtagtctgaaattctaaatggttctctgatttgagggaggttaaacatcaaacaggtttcctctattggccataacatgtataaaatgtgtgttaaggaggaattacaacgtactttgatttgaatactagtagaaactggccaggaaaaaggtacatttttctaaaaattaatggatcacttgggaattactgacttgactagaagtatcaaaggatgtttgcatgtgaatgtgggttatgttctttcccaccttgtagcatattcgatgaaagttgagttaactgatagctaaaaatctgttttaacagcatgtaaaaagttattttatctgttaaaagtcattatacagttttgaatgttatgtagtttctttttaacagtttaggtaataaggtctgttttcattctggtgcttttattaattttgatagtatgatgttacttactactgaaatgtaagctagagtgtacactagaatgtaagctccatgagagcaggtaccttgtctgtcttctctgctgtatctattcccaacgcttgatgatggtgcctggcacatagtaggcactcaataaatatttgttgaatgaatgaa

SEQ ID NO: 4 - protein, 694 aa, Homo sapiens
MPSATSHSGSGSKSSGPPPPSGSSGSEAAAGAGAAAPASQHPATGTGAVQTEAMKQILGVIDKKLRNLEKKKGKLDDYQERMNKGERLNQDQLDAVSKYQEVTNNLEFAKELQRSFMALSQDIQKTIKKTARREQLMREEAEQKRLKTVLELQYVLDKLGDDEVRTDLKQGLNGVPILSEEELSLLDEFYKLVDPERDMSLRLNEQYEHASIHLWDLLEGKEKPVCGTTYKVLKEIVERVFQSNYFDSTHNHQNGLCEEEEAASAPAVEDQVPEAEPEPAEEYTEQSEVESTEYVNRQFMAETQFTSGEKEQVDEWTVETVEVVNSLQQQPQAASPSVPEPHSLTPVAQADPLVRRQRVQDLMAQMQGPYNFIQDSMLDFENQTLDPAIVSAQPMNPTQNMDMPQLVCPPVHSESRLAQPNQVPVQPEATQVPLVSSTSEGYTASQPLYQPSHATEQRPQKEPIDQIQATISLNTDQTTASSSLPAASQPQVFQAGTSKPLHSSGINVNAAPFQSMQTVFNMNAPVPPVNEPETLKQQNQYQASYNQSFSSQPHQVEQTELQQEQLQTVVGTYHGSPDQSHQVTGNHQQPPQQNTGFPRSNQPYYNSRGVSRGGSRGARGLMNGYRGPANGFRGGYDGYRPSFSNTPNSGYTQSQFSAPRDYSGYQRDGYQQNFKRGSGQSGPRGAPRGNILWW

SEQ ID NO: 5 - DNA, 1605 bp, Canis familiaris
  CDS (46)..(1392)
gtcacaaataacttggagtttgcaaaagaattacagaggagtttcatggcattaagtcaagatattcagaaaacaataaagaagactgcacgtcgggagcagcttatgagagaggaagcggaacaaaaacgtttaaaaactgtacttgagctccagtatgttttggacaaattgggagatgatgaagtgagaactgacctgaagcaaggtttgaatggagtgccaatattgtctgaagaagaattgtcgttgttggatgaattctacaaattagcagaccctgaacgggacatgagcttgaggttgaatgagcagtatgaacatgcttccattcacctgtgggacttgctggaaggaaaggaaaagtctgtatgtggaacaacctataaagcactaaaggaaattgttgagcgtgttttccagtcaaattactttgacagcactcacaaccaccagaatgggctatgtgaggaagaagaggcagcctcagcacctacagttgaagaccaggtagctgaagctgagcctgagccagcagaagaatacactgaacaaagtgaagttgaatcaacagagtatgtaaatagacaatttatggcagaaacacagttcagcagtggtgaaaaggagcaggtagatgagtggacggtcgaaacagtggaggtggtgaattcactccagcagcaacctcaggctgcgtctccttcagtaccagagccccactctttgactccggtggctcaggcagatccccttgtgagaagacagcgagtccaggaccttatggcgcagatgcaggggccctataatttcatacaggattcaatgctggattttgaaaaccagacactcgatcctgccattgtatctgcacagcctatgaatccgacacaaaacatggacatgccccagctggtttgccctccagttcattctgaatctagacttgctcaacctaatcaagttcctgtacaaccagaagctacacaggttcctttggtttcatccacaagtgaggggtatacagcatctcaacccttgtaccagccttctcatgctacagagcaacgaccacaaaaggaaccaattgaccagattcaggcaacaatctctttaaatacagaccagactacagcgtcatcatcccttccggctgcttctcagcctcaggtattccaggctgggacaagcaaaccattacatagcagtggaatcaatgtaaatgcagctccattccaatccatgcaaacggtgttcaatatgaatgccccagttcctcctgttaatgaaccagaaactttgaaacaacaaaatcagtaccaggccagttataaccagagcttttctagtcagcctcaccaagtagaacaaacagagggatgccgcaaatgaacactcagcaagtgaattaatctgattcacaggattatgtttaaacgccaaaaacacactggccagtgtaccataatatgttaccagaagagttattatctatttgttctccctttcaggaaacttattgtaaagggactgttttcatcccataaagacaggactacaattgtcagctttatattacctggaaaaaaaaaaaaaaaaaaaaaa

SEQ ID NO: 6 - protein, 448 aa, Canis familiaris
MALSQDIQKTIKKTARREQLMREEAEQKRLKTVLELQYVLDKLGDDEVRTDLKQGLNGVPILSEEELSLLDEFYKLADPERDMSLRLNEQYEHASIHLWDLLEGKEKSVCGTTYKALKEIVERVFQSNYFDSTHNHQNGLCEEEEAASAPTVEDQVAEAEPEPAEEYTEQSEVESTEYVNRQFMAETQFSSGEKEQVDEWTVETVEVVNSLQQQPQAASPSVPEPHSLTPVAQADPLVRRQRVQDLMAQMQGPYNFIQDSMLDFENQTLDPAIVSAQPMNPTQNMDMPQLVCPPVHSESRLAQPNQVPVQPEATQVPLVSSTSEGYTASQPLYQPSHATEQRPQKEPIDQIQATISLNTDQTTASSSLPAASQPQVFQAGTSKPLHSSGINVNAAPFQSMQTVFNMNAPVPPVNEPETLKQQNQYQASYNQSFSSQPHQVEQTEGCRK

SEQ ID NO: 7 - DNA, 4154 bp, Canis familiaris
  CDS (1)..(2154)
atgccgtcggccaccagcctcagcggaagcggcagcaagtcgtcgggcccgccgcccccgtcgggttcctccgggagcgaggcggcggcggcggcgggggcggcgggggcggcgggggccggggcggctgcgcccgcctcccagcaccccgcgaccggcaccggcgctgtccagaccgaggccatgaagcagatcctcggggtgatcgacaagaaactccggaacctggagaagaaaaagggcaagcttgatgattaccaggaacgaatgaacaaaggggaaaggcttaatcaagatcagctggatgccgtatctaagtaccaggaagtcacaaataacttggagtttgcaaaagaattacagaggagtttcatggcattaagtcaagatattcagaaaacaataaagaagactgcacgtcgggagcagcttatgagagaggaagcggaacaaaaacgtttaaaaactgtacttgagctccagtatgttttggacaaattgggagatgatgaagtgagaactgacctgaagcaaggtttgaatggagtgccaatattgtctgaagaagaattgtcgttgttggatgaattctacaaattagcagaccctgaacgggacatgagcttgaggttgaatgagcagtatgaacatgcttccattcacctgtgggacttgctggaaggaaaggaaaagtctgtatgtggaacaacctataaagcactaaaggaaattgttgagcgtgttttccagtcaaattactttgacagcactcacaaccaccagaatgggctatgtgaggaagaagaggcagcctcagcacctacagttgaagaccaggtagctgaagctgagcctgagccagcagaagaatacactgaacaaagtgaagttgaatcaacagagtatgtaaatagacaatttatggcagaaacacagttcagcagtggtgaaaaggagcaggtagatgagtggacggtcgaaacagtggaggtggtgaattcactccagcagcaacctcaggctgcgtctccttcagtaccagagccccactctttgactccggtggctcaggcagatccccttgtgagaagacagcgagtccaggaccttatggcgcagatgcaggggccctataatttcatacaggattcaatgctggattttgaaaaccagacactcgatcctgccattgtatctgcacagcctatgaatccgacacaaaacatggacatgccccagctggtttgccctccagttcattctgaatctagacttgctcaacctaatcaagttcctgtacaaccagaagctacacaggttcctttggtttcatccacaagtgaggggtatacagcatctcaacccttgtaccagccttctcatgctacagagcaacgaccacaaaaggaaccaattgaccagattcaggcaacaatctctttaaatacagaccagactacagcgtcatcatcccttccggctgcttctcagcctcaggtattccaggctgggacaagcaaaccattacatagcagtggaatcaatgtaaatgcagctccattccaatccatgcaaacggtgttcaatatgaatgccccagttcctcctgttaatgaaccagaaactttgaaacaacaaaatcagtaccaggccagttataaccagagcttttctagtcagcctcaccaagtagaacaaacagaccttcagcaagaacagcttcaaacagtggttggcacttaccatggttcccaggaccagccccaccaagtgactggtaaccatcagcagcctccccagcagaacactggatttccacgtagcagtcagccctattacaatagtcgtggtgtgtctcgtggtggttcccgtggtgctagaggcttaatgaatggatacaggggccctgccaatggattcagaggaggatatgatggttaccgcccttcattctctaacactccaaacagtggttatacacagtctcagttcagtgctccccgggactactctggctatcagcgggatggatatcagcagaatttcaagcgaggctctgggcagagtggaccacggggagccccacgaggtcgtggagggcccccaagacccaacagagggatgccgcaaatgaacactcagcaagtgaattaatctgattcacaggattatgtttaaacgccaaaaacacactggccagtgtaccataatatgttaccagaagagttattatctatttgttctccctttcaggaaacttattgtaaagggactgttttcatcccataaagacaggactacaattgtcagctttatattacctggatatggaaggaaactatttttattctgcatgttcttcctaagcgtcatcttgagccttgcacatgatactcagattcctcacccttgcttaggagtaaaacataatacactttacagggtgatatctccatagttatttgaagtggcttggaaaaagcaagattaacttctgacattggataaaaatcaacaaatcagccctagagttattcaaatggtaattgacaaaaactaaaatatttcccttcgagaaggagtggaatgtggtttggcagaacaactgcatttcacagcttttccggttaaattggagcactaaacgtttagatgcataccaaattatgcatgggcccttaatataaaaggctggctaccagctttgacacagcactattcatcctctggccaaacaactgtggttaaacaacacatgtaaattgctttttaacagctgatactataataagacaaagccaaaatgcaaaaattgggctttgattggcactttttgaaaaatatgcaacaaatatgggatgtaatctggatggccgcttctgtacttaatgtgaagtatttagatacctttttgaacacttaacagtttcttctgacaatgacttttgtaaggattggtactatctatcattccttataatgtacattgtctgtcactaatcctcagatcttgctgtattgtcacctaaattggtacaggtactgatgaaaatatctaatggataatcataacactcttggtcacatgtttttcctgcagcctgaaggtttttaaaagaaaaagatatcaaatgcctgctgctaccacccttttaaattgctatcttttgaaaagcaccagtatgtgttttagattgatttccctattttagggaaatgacagacagtagtttcagttctgatggtataagcaaaacaaataaaacatgtttataaaagttgtatcttgaaacactggtgttcaacagctagcagcttatgtggttcaccccatgcattgttagtgtttcagattttatggttatctccagcagctgtttctgtagtacttgcatttatcttttgtctaaccctaatattctcacggaggcatttatattcaaagtggtgatcccttcacttagacgcatagggagagtcacaagtttgatgaagaggacagtgtagtaatttatatgctgttggaatttgtgctagcagtttgagcactagttctgtgtgcctatgaacttaatgctgcttgtcatattccactttgacttcatggagaattaatcccatctactcagcaaaggctatactaatactaagttaatggtattttctgtgcagaaattgaattttgttttattagcatttagctaaggaatttttccagtaggtgctcagctactaaagaaaaacaaaaacaagacacaaaactattctcaaacattcattgttagacaactggagtttttgctggttttgtaacctactaaaatggataggctgttgaacattccacattcaaaagttttttgtagggtggtggggaagggggggtgtcttcaatgtttattttaaaataaaataagttcttgacttttctcatgtgtggttgtggtacatcatattggaagggttatctgtttacttttgcaaatgagtatttctcttgctagcacctcccgttgtgcgctttaaatgacatctgcctgggatgtaccacaaccatatgttagctgtattttatggggaatagataaaatattcgtggtttattgggtaatccctagatgtgtatgcttacaatcctatatataaaactaaat

SEQ ID NO: 8 - protein, 717 aa, Canis familiaris
MPSATSLSGSGSKSSGPPPPSGSSGSEAAAAAGAAGAAGAGAAAPASQHPATGTGAVQTEAMKQILGVIDKKLRNLEKKKGKLDDYQERMNKGERLNQDQLDAVSKYQEVTNNLEFAKELQRSFMALSQDIQKTIKKTARREQLMREEAEQKRLKTVLELQYVLDKLGDDEVRTDLKQGLNGVPILSEEELSLLDEFYKLADPERDMSLRLNEQYEHASIHLWDLLEGKEKSVCGTTYKALKEIVERVFQSNYFDSTHNHQNGLCEEEEAASAPTVEDQVAEAEPEPAEEYTEQSEVESTEYVNRQFMAETQFSSGEKEQVDEWTVETVEVVNSLQQQPQAASPSVPEPHSLTPVAQADPLVRRQRVQDLMAQMQGPYNFIQDSMLDFENQTLDPAIVSAQPMNPTQNMDMPQLVCPPVHSESRLAQPNQVPVQPEATQVPLVSSTSEGYTASQPLYQPSHATEQRPQKEPIDQIQATISLNTDQTTASSSLPAASQPQVFQAGTSKPLHSSGINVNAAPFQSMQTVFNMNAPVPPVNEPETLKQQNQYQASYNQSFSSQPHQVEQTDLQQEQLQTVVGTYHGSQDQPHQVTGNHQQPPQQNTGFPRSSQPYYNSRGVSRGGSRGARGLMNGYRGPANGFRGGYDGYRPSFSNTPNSGYTQSQFSAPRDYSGYQRDGYQQNFKRGSGQSGPRGAPRGRGGPPRPNRGMPQMNTQQVN

SEQ ID NO: 9 - DNA, 4939 bp, Canis familiaris
  CDS (1)..(2109)
atgccgtcggccaccagcctcagcggaagcggcagcaagtcgtcgggcccgccgcccccgtcgggttcctccgggagcgaggcggcggcggcggcgggggcggcgggggcggcgggggccggggcggctgcgcccgcctcccagcaccccgcgaccggcaccggcgctgtccagaccgaggccatgaagcagatcctcggggtgatcgacaagaaactccggaacctggagaagaaaaagggcaagcttgatgattaccaggaacgaatgaacaaaggggaaaggcttaatcaagatcagctggatgccgtatctaagtaccaggaagtcacaaataacttggagtttgcaaaagaattacagaggagtttcatggcattaagtcaagatattcagaaaacaataaagaagactgcacgtcgggagcagcttatgagagaggaagcggaacaaaaacgtttaaaaactgtacttgagctccagtatgttttggacaaattgggagatgatgaagtgagaactgacctgaagcaaggtttgaatggagtgccaatattgtctgaagaagaattgtcgttgttggatgaattctacaaattagcagaccctgaacgggacatgagcttgaggttgaatgagcagtatgaacatgcttccattcacctgtgggacttgctggaaggaaaggaaaagtctgtatgtggaacaacctataaagcactaaaggaaattgttgagcgtgttttccagtcaaattactttgacagcactcacaaccaccagaatgggctatgtgaggaagaagaggcagcctcagcacctacagttgaagaccaggtagctgaagctgagcctgagccagcagaagaatacactgaacaaagtgaagttgaatcaacagagtatgtaaatagacaatttatggcagaaacacagttcagcagtggtgaaaaggagcaggtagatgagtggacggtcgaaacagtggaggtggtgaattcactccagcagcaacctcaggctgcgtctccttcagtaccagagccccactctttgactccggtggctcaggcagatccccttgtgagaagacagcgagtccaggaccttatggcgcagatgcaggggccctataatttcatacaggattcaatgctggattttgaaaaccagacactcgatcctgccattgtatctgcacagcctatgaatccgacacaaaacatggacatgccccagctggtttgccctccagttcattctgaatctagacttgctcaacctaatcaagttcctgtacaaccagaagctacacaggttcctttggtttcatccacaagtgaggggtatacagcatctcaacccttgtaccagccttctcatgctacagagcaacgaccacaaaaggaaccaattgaccagattcaggcaacaatctctttaaatacagaccagactacagcgtcatcatcccttccggctgcttctcagcctcaggtattccaggctgggacaagcaaaccattacatagcagtggaatcaatgtaaatgcagctccattccaatccatgcaaacggtgttcaatatgaatgccccagttcctcctgttaatgaaccagaaactttgaaacaacaaaatcagtaccaggccagttataaccagagcttttctagtcagcctcaccaagtagaacaaacagaccttcagcaagaacagcttcaaacagtggttggcacttaccatggttcccaggaccagccccaccaagtgactggtaaccatcagcagcctccccagcagaacactggatttccacgtagcagtcagccctattacaatagtcgtggtgtgtctcgtggtggttcccgtggtgctagaggcttaatgaatggatacaggggccctgccaatggattcagaggaggatatgatggttaccgcccttcattctctaacactccaaacagtggttatacacagtctcagttcagtgctccccgggactactctggctatcagcgggatggatatcagcagaatttcaagcgaggctctgggcagagtggaccacggggagccccacgaggtaatattttgtggtggtgatcctagctcctaagtggagcttctgttctggccttggaagagctgttccatagtctgcatgtaggttacatgttaggaatacatttatcattaccagacttgttgctagggattaaatgaaatgctctgtttctaaaacttctcttgaacccaaatttaattttttgaatgactttccctgttactatataaattgtcttgaaaactagaacatttctcctcctcagaaaaagtgtttttccaactgcaaattatttttcaggtcctaaaacctgctaaatgtttttaggaagtacttactgaaacatttttgtaagacatttttggaatgagattgaacatttatataaatttattattattcctctttcatttttgaacatgcatattatattttagggtcagaaatcctttaatggccaaataagccatagttacatttagagaaccatttagaagtgatagaactaactgaaatttcaatgcctttggatcattaatagcgatataaatttcaaattgtttctgacttttaaataaaacatccaaaatcctaactaacttcctgaactatatttaaaaattacaggtttaaggagtttctggttttttttctcttaccataggaaaactgtttcctgtttggccaggaagtcaacctgtgtaataattagaagtagcatttcatatgatctgaagttctaaatggttctctgatttaagggaagttaaattgaataggtttcctctagttattggccataacatgtataaaatgtatattaaggaggaatacaaagtactttgatttcaatgctagtagaaactggccagcaaaaaggtgcattttatttttaaattaatggatcacttgggaattactgacttgaagtatcaaaggatatttgcatgtgaatgtgggttatgttctttctcaccttgtagcatattctatgaaagttgagttgactggtagctaaaaatctgttttaacagcatgtaaaaagttattttatctgttacaagtcattatacaattttgaatgttatgtagtttctttttaacagtttaggtaacaaggtctgtttttcattctggtgcttttattaattttgatagtatgatgttacttactactgaaatgtaagctagagtgtacactagaatgtaagctccatgagagcaggtaccttgtctgtcttcactgctgtatctatttccaacgcctgatgacagtgcctgacacatagtaggcactcaataaatacttgttgaatgaatgaatgaatgagtactggtggaatactccattagctctactcttcttttagctagagaacatgagcaaatttgcgcatgacaacttccaggacaggtgaacactgaagaattgacctcttaaacctaataatgtggtgacaagctgcccacatgcttcttgacttcagatgaaaatctgcttgaaggcaaagcaaataatatttgaaagaaaaaccaaatgccatttttgtcttctaggtcgtggagggcccccaagacccaacagagggatgccgcaaatgaacactcagcaagtgaattaatctgattcacaggattatgtttaaacgccaaaaacacactggccagtgtaccataatatgttaccagaagagttattatctatttgttctccctttcaggaaacttattgtaaagggactgttttcatcccataaagacaggactacaattgtcagctttatattacctggatatggaaggaaactatttttattctgcatgttcttcctaagcgtcatcttgagccttgcacatgatactcagattcctcacccttgcttaggagtaaaacataatacactttacagggtgatatctccatagttatttgaagtggcttggaaaaagcaagattaacttctgacattggataaaaatcaacaaatcagccctagagttattcaaatggtaattgacaaaaactaaaatatttcccttcgagaaggagtggaatgtggtttggcagaacaactgcatttcacagcttttccggttaaattggagcactaaacgtttagatgcataccaaattatgcatgggcccttaatataaaaggctggctaccagctttgacacagcactattcatcctctggccaaacaactgtggttaaacaacacatgtaaattgctttttaacagctgatactataataagacaaagccaaaatgcaaaaattgggctttgattggcactttttgaaaaatatgcaacaaatatgggatgtaatctggatggccgcttctgtacttaatgtgaagtatttagatacctttttgaacacttaacagtttcttctgacaatgacttttgtaaggattggtactatctatcattccttataatgtacattgtctgtcactaatcctcagatcttgctgtattgtcacctaaattggtacaggtactgatgaaaatatctaatggataatcataacactcttggtcacatgtttttcctgcagcctgaaggtttttaaaagaaaaagatatcaaatgcctgctgctaccacccttttaaattgctatcttttgaaaagcaccagtatgtgttttagattgatttccctattttagggaaatgacagacagtagtttcagttctgatggtataagcaaaacaaataaaacatgtttataaaagttgtatcttgaaacactggtgttcaacagctagcagcttatgtggttcaccccatgcattgttagtgtttcagattttatggttatctccagcagctgtttctgtagtacttgcatttatc

SEQ ID NO: 10 - protein, 702 aa, Canis familiaris
MPSATSLSGSGSKSSGPPPPSGSSGSEAAAAAGAAGAAGAGAAAPASQHPATGTGAVQTEAMKQILGVIDKKLRNLEKKKGKLDDYQERMNKGERLNQDQLDAVSKYQEVTNNLEFAKELQRSFMALSQDIQKTIKKTARREQLMREEAEQKRLKTVLELQYVLDKLGDDEVRTDLKQGLNGVPILSEEELSLLDEFYKLADPERDMSLRLNEQYEHASIHLWDLLEGKEKSVCGTTYKALKEIVERVFQSNYFDSTHNHQNGLCEEEEAASAPTVEDQVAEAEPEPAEEYTEQSEVESTEYVNRQFMAETQFSSGEKEQVDEWTVETVEVVNSLQQQPQAASPSVPEPHSLTPVAQADPLVRRQRVQDLMAQMQGPYNFIQDSMLDFENQTLDPAIVSAQPMNPTQNMDMPQLVCPPVHSESRLAQPNQVPVQPEATQVPLVSSTSEGYTASQPLYQPSHATEQRPQKEPIDQIQATISLNTDQTTASSSLPAASQPQVFQAGTSKPLHSSGINVNAAPFQSMQTVFNMNAPVPPVNEPETLKQQNQYQASYNQSFSSQPHQVEQTDLQQEQLQTVVGTYHGSQDQPHQVTGNHQQPPQQNTGFPRSSQPYYNSRGVSRGGSRGARGLMNGYRGPANGFRGGYDGYRPSFSNTPNSGYTQSQFSAPRDYSGYQRDGYQQNFKRGSGQSGPRGAPRGNILWW

SEQ ID NO: 11 - DNA, 3306 bp, Canis familiaris
  CDS (1)..(2040)
atgccgtcggccaccagcctcagcggaagcggcagcaagtcgtcgggcccgccgcccccgtcgggttcctccgggagcgaggcggcggcggcggcgggggcggcgggggcggcgggggccggggcggctgcgcccgcctcccagcaccccgcgaccggcaccggcgctgtccagaccgaggccatgaagcagatcctcggggtgatcgacaagaaactccggaacctggagaagaaaaagggcaagcttgatgattaccaggaacgaatgaacaaaggggaaaggcttaatcaagatcagctggatgccgtatctaagtaccaggaagtcacaaataacttggagtttgcaaaagaattacagaggagtttcatggcattaagtcaagatattcagaaaacaataaagaagactgcacgtcgggagcagcttatgagagaggaagcggaacaaaaacgtttaaaaactgtacttgagctccagtatgttttggacaaattgggagatgatgaagtgagaactgacctgaagcaaggtttgaatggagtgccaatattgtctgaagaagaattgtcgttgttggatgaattctacaaattagcagaccctgaacgggacatgagcttgaggttgaatgagcagtatgaacatgcttccattcacctgtgggacttgctggaaggaaaggaaaagtctgtatgtggaacaacctataaagcactaaaggaaattgttgagcgtgttttccagtcaaattactttgacagcactcacaaccaccagaatgggctatgtgaggaagaagaggcagcctcagcacctacagttgaagaccaggtagctgaagctgagcctgagccagcagaagaatacactgaacaaagtgaagttgaatcaacagagtatgtaaatagacaatttatggcagaaacacagttcagcagtggtgaaaaggagcaggtagatgagtggacggtcgaaacagtggaggtggtgaattcactccagcagcaacctcaggctgcgtctccttcagtaccagagccccactctttgactccggtggctcaggcagatccccttgtgagaagacagcgagtccaggaccttatggcgcagatgcaggggccctataatttcatacaggattcaatgctggattttgaaaaccagacactcgatcctgccattgtatctgcacagcctatgaatccgacacaaaacatggacatgccccagctggtttgccctccagttcattctgaatctagacttgctcaacctaatcaagttcctgtacaaccagaagctacacaggttcctttggtttcatccacaagtgaggggtatacagcatctcaacccttgtaccagccttctcatgctacagagcaacgaccacaaaaggaaccaattgaccagattcaggcaacaatctctttaaatacagaccagactacagcgtcatcatcccttccggctgcttctcagcctcaggtattccaggctgggacaagcaaaccattacatagcagtggaatcaatgtaaatgcagctccattccaatccatgcaaacggtgttcaatatgaatgccccagttcctcctgttaatgaaccagaaactttgaaacaacaaaatcagtaccaggccagttataaccagagcttttctagtcagcctcaccaagtagaacaaacagaccttcagcaagaacagcttcaaacagtggttggcacttaccatggttcccaggaccagccccaccaagtgactggtaaccatcagcagcctccccagcagaacactggatttccacgtagcagtcagccctattacaatagtcgtggtgtgtctcgtggtggttcccgtggtgctagaggcttaatgaatggatacaggggccctgccaatggattcagaggaggatatgatggttaccgcccttcattctctaacactccaaacagtggttatacacagtctcagttcagtgctccccgggactactctggctatcagcggggatgccgcaaatgaacactcagcaagtgaattaatctgattcacaggattatgtttaaacgccaaaaacacactggccagtgtaccataatatgttaccagaagagttattatctatttgttctccctttcaggaaacttattgtaaagggactgttttcatcccataaagacaggactacaattgtcagctttatattacctggatatggaaggaaactatttttattctgcatgttcttcctaagcgtcatcttgagccttgcacatgatactcagattcctcacccttgcttaggagtaaaacataatacactttacagggtgatatctccatagttatttgaagtggcttggaaaaagcaagattaacttctgacattggataaaaatcaacaaatcagccctagagttattcaaatggtaattgacaaaaactaaaatatttcccttcgagaaggagtggaatgtggtttggcagaacaactgcatttcacagcttttccggttaaattggagcactaaacgtttagatgcataccaaattatgcatgggcccttaatataaaaggctggctaccagctttgacacagcactattcatcctctggccaaacaactgtggttaaacaacacatgtaaattgctttttaacagctgatactataataagacaaagccaaaatgcaaaaattgggctttgattggcactttttgaaaaatatgcaacaaatatgggatgtaatctggatggccgcttctgtacttaatgtgaagtatttagatacctttttgaacacttaacagtttcttctgacaatgacttttgtaaggattggtactatctatcattccttataatgtacattgtctgtcactaatcctcagatcttgctgtattgtcacctaaattggtacaggtactgatgaaaatatctaatggataatcataacactcttggtcacatgtttttcctgcagcctgaaggtttttaaaagaaaaagatatcaaatgcctgctgctaccacccttttaaattgctatcttttgaaaagcaccagtatgtgttttagattgatttccctattttagggaaatgacagacagtagtttcagttctgatggtataagcaaaacaaataaaacatgtttataaaagttgtatcttgaaacactggtgttcaacagctagcagcttatgtggttcaccccatgcattgttagtgtttcagattttatggttatctccagcagctgtttctgtagtacttgcatttatc

SEQ ID NO: 12 - protein, 679 aa, Canis familiaris
MPSATSLSGSGSKSSGPPPPSGSSGSEAAAAAGAAGAAGAGAAAPASQHPATGTGAVQTEAMKQILGVIDKKLRNLEKKKGKLDDYQERMNKGERLNQDQLDAVSKYQEVTNNLEFAKELQRSFMALSQDIQKTIKKTARREQLMREEAEQKRLKTVLELQYVLDKLGDDEVRTDLKQGLNGVPILSEEELSLLDEFYKLADPERDMSLRLNEQYEHASIHLWDLLEGKEKSVCGTTYKALKEIVERVFQSNYFDSTHNHQNGLCEEEEAASAPTVEDQVAEAEPEPAEEYTEQSEVESTEYVNRQFMAETQFSSGEKEQVDEWTVETVEVVNSLQQQPQAASPSVPEPHSLTPVAQADPLVRRQRVQDLMAQMQGPYNFIQDSMLDFENQTLDPAIVSAQPMNPTQNMDMPQLVCPPVHSESRLAQPNQVPVQPEATQVPLVSSTSEGYTASQPLYQPSHATEQRPQKEPIDQIQATISLNTDQTTASSSLPAASQPQVFQAGTSKPLHSSGINVNAAPFQSMQTVFNMNAPVPPVNEPETLKQQNQYQASYNQSFSSQPHQVEQTDLQQEQLQTVVGTYHGSQDQPHQVTGNHQQPPQQNTGFPRSSQPYYNSRGVSRGGSRGARGLMNGYRGPANGFRGGYDGYRPSFSNTPNSGYTQSQFSAPRDYSGYQRGCRK

SEQ ID NO: 13 - DNA, 2281 bp, Canis familiaris
  CDS (1)..(2154)
atgccgtcggccaccagcctcagcggaagcggcagcaagtcgtcgggcccgccgcccccgtcgggttcctccgggagcgaggcggcggcggcggcgggggcggcgggggcggcgggggccggggcggctgcgcccgcctcccagcaccccgcgaccggcaccggcgctgtccagaccgaggccatgaagcagatcctcggggtgatcgacaagaaactccggaacctggagaagaaaaagggcaagcttgatgattaccaggaacgaatgaacaaaggggaaaggcttaatcaagatcagctggatgccgtatctaagtaccaggaagtcacaaataacttggagtttgcaaaagaattacagaggagtttcatggcattaagtcaagatattcagaaaacaataaagaagactgcacgtcgggagcagcttatgagagaggaagcggaacaaaaacgtttaaaaactgtacttgagctccagtatgttttggacaaattgggagatgatgaagtgagaactgacctgaagcaaggtttgaatggagtgccaatattgtctgaagaagaattgtcgttgttggatgaattctacaaattagcagaccctgaacgggacatgagcttgaggttgaatgagcagtatgaacatgcttccattcacctgtgggacttgctggaaggaaaggaaaagtctgtatgtggaacaacctataaagcactaaaggaaattgttgagcgtgttttccagtcaaattactttgacagcactcacaaccaccagaatgggctatgtgaggaagaagaggcagcctcagcacctacagttgaagaccaggtagctgaagctgagcctgagccagcagaagaatacactgaacaaagtgaagttgaatcaacagagtatgtaaatagacaatttatggcagaaacacagttcagcagtggtgaaaaggagcaggtagatgagtggacggtcgaaacagtggaggtggtgaattcactccagcagcaacctcaggctgcgtctccttcagtaccagagccccactctttgactccggtggctcaggcagatccccttgtgagaagacagcgagtccaggaccttatggcgcagatgcaggggccctataatttcatacaggattcaatgctggattttgaaaaccagacactcgatcctgccattgtatctgcacagcctatgaatccgacacaaaacatggacatgccccagctggtttgccctccagttcattctgaatctagacttgctcaacctaatcaagttcctgtacaaccagaagctacacaggttcctttggtttcatccacaagtgaggggtatacagcatctcaacccttgtaccagccttctcatgctacagagcaacgaccacaaaaggaaccaattgaccagattcaggcaacaatctctttaaatacagaccagactacagcgtcatcatcccttccggctgcttctcagcctcaggtattccaggctgggacaagcaaaccattacatagcagtggaatcaatgtaaatgcagctccattccaatccatgcaaacggtgttcaatatgaatgccccagttcctcctgttaatgaaccagaaactttgaaacaacaaaatcagtaccaggccagttataaccagagcttttctagtcagcctcaccaagtagaacaaacagaccttcagcaagaacagcttcaaacagtggttggcacttaccatggttcccaggaccagccccaccaagtgactggtaaccatcagcagcctccccagcagaacactggatttccacgtagcagtcagccctattacaatagtcgtggtgtgtctcgtggtggttcccgtggtgctagaggcttaatgaatggatacaggggccctgccaatggattcagaggaggatatgatggttaccgcccttcattctctaacactccaaacagtggttatacacagtctcagttcagtgctccccgggactactctggctatcagcgggatggatatcagcagaatttcaagcgaggctctgggcagagtggaccacggggagccccacgaggtcgtggagggcccccaagacccaacagagggatgccgcaaatgaacactcagcaagtgaattaatctgattcacaggattatgtttaaacgccaaaaacacactggccagtgtaccataatatgttaccagaagagttattatctatttggactgttttcatcccataaagacaggactacaattgtcagc

SEQ ID NO: 14 - protein, 717 aa, Canis familiaris; identical to SEQ ID NO: 8

SEQ ID NO: 15 - DNA, 3386 bp, Bos taurus
  CDS (82)..(2208)
cgcgtctcgccccgtccaccgattgactcgccgctcttgtccttcctcccgctctttcttctctccccttacggtttcaagatgccttcggccaccagccacagcggaagcggcagcaagtcgtccggaccgccaccgccgtcgggttcctccgggaatgaggcgggggccggggccgccgcgccggcttcccaacaccccatgaccggcaccggggctgtccagaccgaggccatgaagcagattctcggggtgatcgacaagaaacttcggaacctggagaagaaaaagggcaagcttgatgattatcaggaacgaatgaacaaaggggaaaggcttaatcaagatcagctggatgccgtgtctaagtaccaggaagtcacaaataacttggagtttgcaaaagaattacagaggagtttcatggcattaagccaagatattcagaaaacaataaagaagacagcacgtcgggagcagcttatgagagaggaagctgaacagaaacgtttaaaaacagtacttgagctgcagtatgttttggacaaactaggagatgatgaagtgagaactgacctgaagcaaggtttgaatggagtgccaatattgtctgaagaggagttgtcgttgttagatgagttctacaaattagcagaccctgaacgagacatgagcttgaggttgaatgagcagtatgaacatgcctccattcacctgtgggacttgctggaaggaaaggaaaaacctgtatgtggaacaacttataaagctctaaaggaaattgttgagcgtgttttccagtcaaactactttgacagcacccacaaccaccagaatggtctgtgtgaggaagaggaggcagcctcagcacctacagttgaagaccaggcagctgaagctgaacctgagccagtggaagaatatactgaacaaaatgaggttgaatcaacagagtatgtaaatagacaatttatggcagaaacacagttcagcagtggtgaaaaggagcaggtagatgattggacagttgaaacagttgaggtggtaaattcactccagcagcaacctcaggctgcatctccttcagtaccagaaccccactctttgaccccagtggctcaagccgatcccctcgtgagaagacagcgagtacaggaccttatggcacaaatgcaggggccctataatttcatacaggattcaatgttggattttgaaaaccagacacttgatcctgccattgtatctgcacagccgatgaatccagcacagaacatggacataccccagctggtttgccctccagttcattctgaatctagacttgctcaacctaatcaagtttctgtacagccagaagctacacaggttcctttggtttcatccacaagtgagggatatacagcatctcaacccttgtaccaaccttctcatgctactgaccaacgaccacaaaaggaaccgattgatcagattcaggcgacgatctctttaaatacagaccagactacagcatcatcatcccttcctgctgcttctcagcctcaagtgttccaggctgggacaagcaaacctttacatagcagtggaatcaatgtaaatgcagctccattccaatccatgcaaacggtattcaatatgaatgccccagttcctcctgttaatgaaccagaaactttaaaacagcaaaatcagtaccaggccagttacaaccagagcttttccagtcagcctcaccaagtagaacaaacagagcttcagcaagaacagcttcaaacagtggttggcacttatcatggttctcaggaccagccccatcaagtgactggtaaccaccagcagcctcctcagcagaacactggatttccacgtagcaatcagccctattacaacagtcgtggtgtgtctcgtggaggttcccgtggtgctagaggcttgatgaatggatacagaggacctgctaatggattcagaggaggatatgatggttaccgcccttcattctctactaacactccaaacagtggttatacacaatctcaattcagtgctccccgggactactctggctatcagcgggatggatatcagcagaatttcaagcgaggctctgggcagagtggaccacggggagccccacgaggtcgtggagggcccccaagacccaacagagggatgccgcaaatgaacactcagcaagtgaattaatctgattcacaggattatgtttaatcgccaaaaacacactggccagtgtaccataatatgttaccagaagagttattatctatttgttctccctttcaggaaacttattgtaaagggactgttttcatcccataaagacaggactacaattgtcagctttatattacctggatatggaaggaaactatttttactctgcatgttctgtcctaagcgtcatcttgagccttgcacatgatactcagattcctcacccttgcttaggagtaaaacataatatactttaatggggtgatatctccatagttatttgaagtggcttggataaagcaagactgacttctgacattggataaaatctacaaatcagccctagagtcattcagtggtaactgacaaaactaaaatatttcccttgaaaggaagatggaaggagtggagtgtggtttggcagaacaactgcatttcacagcttttccacttaaattggagcactgaacatttagatgcataccgaattatgcatgggccctaatcacacagacaaggctggtgccagccttaggcttgacacggcagtgttcaccctctggccagacgactgtggttcaagacacatgtaaattgctttttaacagctgatactgtataagacaaagccaaaatgcaaaattaggctttgattggcacttttcgaaaaatatgcaacaattaagggatataatctggatggccgcttctgtacttaatgtgaaatatttagatacctttcaaacacttaacagtttctttgacaatgagttttgtaaggattggtagtaaatatcattccttatgacgtacattgtctgtcactaatccttggatcttgctgtattgtcacctaaattggtacaggtactgatgaaaatctaatggataatcataacactcttggttacatgtttttcctgcagcctgaaagtttttataagaaaaagacatcaaatgcctgctgctgccacccttttaaattgctatcttttgaaaagcaccagtatgtgttttagattgatttccctattttagggaaatgacagtcagtagtttcacttctgatggtataagcaaacaaataaaacatgtttataaaaaaaaaaaaaaaaaaaaaaaaaaaaaaaaaaaaaaaaaaaaaaaaa

SEQ ID NO: 16 - protein, 708 aa, Bos taurus
MPSATSHSGSGSKSSGPPPPSGSSGNEAGAGAAAPASQHPMTGTGAVQTEAMKQILGVIDKKLRNLEKKKGKLDDYQERMNKGERLNQDQLDAVSKYQEVTNNLEFAKELQRSFMALSQDIQKTIKKTARREQLMREEAEQKRLKTVLELQYVLDKLGDDEVRTDLKQGLNGVPILSEEELSLLDEFYKLADPERDMSLRLNEQYEHASIHLWDLLEGKEKPVCGTTYKALKEIVERVFQSNYFDSTHNHQNGLCEEEEAASAPTVEDQAAEAEPEPVEEYTEQNEVESTEYVNRQFMAETQFSSGEKEQVDDWTVETVEVVNSLQQQPQAASPSVPEPHSLTPVAQADPLVRRQRVQDLMAQMQGPYNFIQDSMLDFENQTLDPAIVSAQPMNPAQNMDIPQLVCPPVHSESRLAQPNQVSVQPEATQVPLVSSTSEGYTASQPLYQPSHATDQRPQKEPIDQIQATISLNTDQTTASSSLPAASQPQVFQAGTSKPLHSSGINVNAAPFQSMQTVFNMNAPVPPVNEPETLKQQNQYQASYNQSFSSQPHQVEQTELQQEQLQTVVGTYHGSQDQPHQVTGNHQQPPQQNTGFPRSNQPYYNSRGVSRGGSRGARGLMNGYRGPANGFRGGYDGYRPSFSTNTPNSGYTQSQFSAPRDYSGYQRDGYQQNFKRGSGQSGPRGAPRGRGGPPRPNRGMPQMNTQQVN

SEQ ID NO: 17 - DNA, 3150 bp, Equus caballus
  CDS (1)..(1917)
atggagggcaagctcgatgattaccaagagcgaatgaacaaaggagaaaggcttaatcaggatcagctggatgctgtgtctaagtaccaggaagtcacaaataacttggagtttgcgaaagaattgcagaggagtttcatggcgttgagtcaggatattcagaaaacaataaagaagacggcacgtcgggagcagcttatgagagaagaagctgaacagaaacgtttaaaaactgtacttgagctgcagtatgttttggacaaattgggagatgaagaagtgcgaactgacctgaaacaaggtttgaatggagtgccaatactctctgaagaagagttgtcgctgttggatgagttctacaagttagcagaccctgtacgggacatgagcttgaggttgaatgagcagtatgagcatgcctccattcacctgtgggacttgctggaagggaaggaaaaatctgtctgtggaacaacctataaagctctgagggaaattgttgagcgtgttttccagtccaactactttgacagcacccacaaccaccagaatgggctctgtgaggaggaagaggctacctcagctccaacagctgaagaccagggagctgaagctgaacctgagccagcagaagaatacactgaacaaagtgaagttgaatcaacagagtatgtaaatagacagtttatggcagaagcgcagttcagtggtgagaaggagcaggtggatgagtggacagtcgagacggtcgaggtggtaaattcactccagcagcaacctcaggctgcatctccttcagtaccggagccccactctttgactccagtggctcaggcagatccccttgtgagaagacagcgagtacaggaccttatggcgcaaatgcaggggccctataatttcatacaggattcaatgctggattttgaaaaccagacacttgatcctgccattgtatctgcacagcctatgaatccagcacagaatatggacatgccccagctggtttgccctccagttcatgctgaatctagacttgctcaacctaatcaagttcctgtacaaccagaagctacacaggttcctttggtttcatccacaagtgaggggtatacagcatctcagcccttgtaccagccttctcatgctacagagcaacgaccgcaaaaggaaccgactgaccagatccaggcaacaatctctttaaatacagaccagactacagcatcatcatcccttcctgctgcttctcagcctcaggtgttccaggctgggacaagcaaacctttacacagcagtgggatcaatgtaaatgcagcgccattccagtccatgcaaacggtgttcaacatgaatgccccggttcctcctgttaatgaaccagaaactttaaaacagcaaaatcagtaccaggccagctataaccagagcttttccagtccgcctcaccaagtagagcagacagagcttccgcaagagcagcttcagacggtggttggtacttaccatgcttcccaagaccagccccatcaagtgaccggtaaccaccagcagcctccccagcagaacactgggtttccacgtagcagtcagccctattacaacagtcgtggtgtgtctcgtggaggctcccgtggtgctagaggcttgatgaatggatacaggggccctgccaatggattcagaggaggatatgatggttaccgcccttcgttctctaacactccaaacagcggttacacacagtctcagttcagtgctccccgggactactctggctatcagcgggatggatatcagcagaatttcaagcgaggctctgggcagagtggaccccggggagccccacgaggtcgtggagggcccccaagacccaacagagggatgccgcaaatgaacactcagcaagtgaattaatctgattcacaggattatctttaatcgccaaaacacactggccagtgtaccataatatgttaccagaagagttattatctatttgttctccctttcaggaaacttattgtaaagggactgttttcatcccataaagacaggactacagttgtcagctttatattacctggatatggaaggaaactatttttactctgcatgttctgtcctaagcgtcatcttgagccttgcacatgatactcagattcctttcccttgcttaggagtaaaacataatatactttatggggtgataatatctccatagttatttgaagtggcttggaaaaagcaagattgacttttgacattggataaaatctacaaatcagccctagagtttcatggtcattcacaaaactaaaatatttcccttgaaaggaagatggaaggactggagtgtggtttggcagaacaactgcatttcacagcttttcctattaaattggagcactgaatgttaaatgcataccaaattatgcatgggcccttaatcacacatacatggctaccagctttgacacagcactattcatcctctggccaaacgactgtggttaaaaacacgtgtaaattgctttttaacagctgatactgtaaaagacaaagctaaaatgcaaaattaggctttcattggcacttttcgaaaaatatgcaacaaatttgggatgtaatctggatggccacttctgtacttaatgtgaagtatttagatacctttttgaacacttaacagtttcttcgacaatgacttttgtaaggattggtagtatatatcattccttatgacatacattgtctgttgctaatccttggatcttgctgtattgtcacctaaattggtacaggtactgatgaaaatctctcatggataaacctaacactcttcgtcacatgtttttcctgcagcctgaaggtttttaaaaggaaaagatatcaaatgcctgctgctaccacccttttaaattgctatcttttgaaaagcaccagtatgtgtttttagattgatttccctattttagggaaatgacagtcagtagtttcagttctgatggtataagcaaagcaaataaaacgtgtttataaaagttgtatcttgaaacactggtgttcaacagctagcagcttctgtggttcaccccctgccttgttagtgttacccatttatggttatctccagcagcaatttctcta

SEQ ID NO: 18 - protein, 638 aa, Equus caballus
MEGKLDDYQERMNKGERLNQDQLDAVSKYQEVTNNLEFAKELQRSFMALSQDIQKTIKKTARREQLMREEAEQKRLKTVLELQYVLDKLGDEEVRTDLKQGLNGVPILSEEELSLLDEFYKLADPVRDMSLRLNEQYEHASIHLWDLLEGKEKSVCGTTYKALREIVERVFQSNYFDSTHNHQNGLCEEEEATSAPTAEDQGAEAEPEPAEEYTEQSEVESTEYVNRQFMAEAQFSGEKEQVDEWTVETVEVVNSLQQQPQAASPSVPEPHSLTPVAQADPLVRRQRVQDLMAQMQGPYNFIQDSMLDFENQTLDPAIVSAQPMNPAQNMDMPQLVCPPVHAESRLAQPNQVPVQPEATQVPLVSSTSEGYTASQPLYQPSHATEQRPQKEPTDQIQATISLNTDQTTASSSLPAASQPQVFQAGTSKPLHSSGINVNAAPFQSMQTVFNMNAPVPPVNEPETLKQQNQYQASYNQSFSSPPHQVEQTELPQEQLQTVVGTYHASQDQPHQVTGNHQQPPQQNTGFPRSSQPYYNSRGVSRGGSRGARGLMNGYRGPANGFRGGYDGYRPSFSNTPNSGYTQSQFSAPRDYSGYQRDGYQQNFKRGSGQSGPRGAPRGRGGPPRPNRGMPQMNTQQVN

SEQ ID NO: 19 - DNA, 6181 bp, Mus musculus
  CDS (179)..(2302)
gctggctggctaagtccctcccgcgccggctcttgtcccactaggagcagctcagagccgcggggacagggcgaagcggcctgcgcccacggagcgcacgtctctgttctcaacgcagcaccacccttgcccccctcggctgcccactccagacgtccagcggctccgcgcgcgcacgatgccctcggccaccagccacagcggaagcggcagcaaatcgtcgggaccgccgccgccgtccggttcctccgggagtgaggcggcggccggggcagctgcgccggcttctcagcatccggcaaccggcaccggcgccgtccagaccgaggccatgaagcagattctcggcgtaatcgacaagaaacttcggaacctggagaagaaaaagggtaaacttgatgattaccaggaacgaatgaataaaggggaaaggctcaatcaagaccagctggatgccgtatctaagtaccaggaagtcacaaataatttggagtttgcaaaggaattacagaggagtttcatggcattaagtcaagatattcagaaaacaataaagaagacagcacgtcgggaacagcttatgagagaagaagcagaacagaagcgcttaaaaactgtacttgagttacagtatgtattggataagctgggagatgatgatgtgagaacagatctgaaacaaggtttgagtggagtgccaatattgtctgaggaggagttgtcattgctggatgagttctacaagctcgtagatcctgagcgtgacatgagtttaaggttaaatgagcagtatgaacatgcctcaattcacttgtgggatttgctggaagggaaagaaaagcctgtgtgtggaacaacctataaagctctaaaggaaattgttgagcgtgttttccagtcaaactactttgatagcactcacaatcatcaaaatgggttgtgtgaggaggaagaggcggcttcagcgcccacagtggaggaccaggtagctgaagctgaacctgagccagcggaagaatacacagagcaaagtgaggttgaatcaacagagtatgtcaataggcagttcatggcagaaacacagttcagcagtggtgagaaggagcaagtggatgagtggacagttgaaacagttgaggttgtaaactcactccagcagcaacctcaggctgcgtccccttcagtcccagagccccactctttgactccagtggctcagtcagatccacttgtgagaaggcagcgtgtacaagatcttatggcacaaatgcaagggccctataatttcatacaggattcaatgttggattttgaaaatcagacgcttgatcctgccattgtatccgcacagcctatgaaccctacccagaacatggatatgcctcagctggtttgccctcaggttcattctgaatctagacttgcccaatctaatcaagttcctgtacaaccagaagccacacaggttcctttggtttcatccacaagtgaggggtatacagcatctcagcccttgtaccagccatctcatgctacggagcagcggccgcagaaagagccaatggatcagattcaggcaacaatatctttgaatacagaccagactacagcatcctcatcccttcctgctgcttctcagcctcaagtgttccaggctgggacaagtaaacctttgcacagcagtggaatcaatgtaaatgcagctccattccagtccatgcaaacggtgttcaatatgaatgctccagtccctcctgctaatgaaccagaaacgttaaaacaacagagtcagtaccaggccacttataaccagagtttttccagtcagcctcaccaagtggaacaaacagagcttcaacaagaccaactgcaaacggtggttggcacttaccatggatcccaggaccagcctcatcaagtgcctggtaaccaccagcaacccccacagcagaacactggctttccacgtagcagtcagccttattacaacagtcgtggggtatctcgaggagggtctcgtggtgccagaggcttgatgaatggatacaggggccctgccaatggatttagaggaggatatgatggttaccgcccttcattctcgaacactccaaacagtggttattcacagtctcagttcactgctccccgggactactctggttaccagcgggatggatatcagcagaatttcaagcgaggctctgggcagagtggaccacggggagccccacgaggtcgtggagggcccccaagacccaacagagggatgccgcaaatgaacactcagcaagtgaattaatgtgatacacaggattatgtttaatcgccaaaaacacactggccagtgtaccataatatgttaccagaagagttattatctatttgttctccctttcaggaaacttattgtaaagggactgttttcatcccataaagacaggactgcaattgtcagctttacattacctggatatggaaggaaactatttttattctgcatgttctgtcctaagcgtcatcttgagccttgcacacaatacaatactcagattcctcacccttgcttaggagtaaaacattatatacttatggggtgataatatctccatagttagttgaagtggcttggaaaaaaaatgcaagattgaatttttgaccttggataaaatctacaatcagccctagaactattcagtggtaattgacaaagttaaagcattttctttgaaaggaagatggaaggagtggagtgtggtttagcaaaactgcatttcatagctttcccattaaattggagcaccgacagattaaaagcataccaaattatgcatgggtccttactcacacaagtgaggctggctaccagccttgacatagcactcactagtcttctggccaaacgactgtgattaaaacacatgtaaattgctctttagtagtggatactgtgtaagacaaagccaaattgcaaatcaggctttgattggctcttctggaaaatatgcatcaaatatgggggataatctggatgggctgctgctgtgctcaatgtgaactatttagatacctttggaacacttaacagtttctctgaacaatgacttacatggggattggtcctgtttgtcattcctcaccataattgcattgtcatcactaatccttggatcttgctgtattgttactcaaattggtaataggtactgatggaaatcgctaatggatggataatcataacacttttggtcacatgttttctcctgcagcctgaaagttcttaaagaaaaagatatcaaatgcctgctgctaccacccttttaaattgctatctttagaaaagcaccggtatgtgttttagattcatttccctgttttagggaaatgacaggcagtagtttcagttctgatggcaaaacaaataaaaacatgtttctaaaagttgtatcttgaaacactggtgttcaacagctagcagctaaagtaattcaacccatgcattgctagtgtcacagcctttggttatgtctagtagctgtttctgaagtattttcatttatcttttgtcaaatttaaccctgtttgaattctctcctttcctcaaggagacacttatgttcaaagtgttgattctttgccttaggtgcatagagagtagacagtttggagatggaaaggttagcagtgacttagccatatgttctgtgttggaatttgtgctagcagtttgagcactagctctgcgtgcctatgaactgaatgctgcttgtcccattccattttatgtcatggagaaataattccacttggtaacacaaaggctaagttaatgttattttctgtacagaaattaaattttacttttagccttttgtaaactttttttttttttttccaagccggtatcagctactcaaaacaattctcagatattcatcattagacaactggagtttttgctggttttgtagcctactaaaactgctgaggctgttgaacattccacattcaaaagttttgtagggtggtggataatggggaagcttcaatgtttattttaaaataaataaaataagttcttgacttttctcatgtgtggttatggtacatcatattggaagggttatctgtttacttttgccaagactattttgccagcacctacacttgtgtgctttaaaagacaactacctgggatgtaccacaaccatatgttaattgtattttattgggatggataaaatgtttgtggtttattggataatccctagatggtgtgttacgtgtgtagaatataattttatgatagtaagaaagcaaaattgaagaaaataagtttagtattgaatttgagttctgaagtgaattcagggaatgtctcacgtttcgggcttctacccaaagtgtagggcagaaggtgtaaaagttgtttgtagtttgacttgtttattttttaagttgcttattcctttcaacagcaacatatcattagctgtcattctaccattgcagttctagtgagttttaacgtctgcattcaagactgttttaaaagcaacctcactggacagagaactgctaaagtcttttccttaagatctgagtctttgttactcagtatcttctataatatgcaaatgcttgtctagaggcagaagaccttttgtttggtcaagtgtgtattttaccagagtacagggaactgatggtcctacatgtctcttagtgtagtaagactataaaatcttttgtacatgcacaattcacagtatgtttagataccacgtgtataatgcccccccctcccccaggtagcatgccattgatgactttttgcttagggccattttattaccagggccttaatattcctaaaaagatgattttttttcatcctttctcctcttttgatcattgtatcttgatattaaaaacatgaccttccaatgattgtagtaaattaacttctatagttcttttgtctctatatgtattcatatatatgctattgtatagagacttcaaggagacatggagatgcatgcttattctcaggttcattcactaaggtgcttggcagacaaccagtttctaagtgcagaatgtagttaagcagcttcatatatgtgccaggcaatttgttttgttaaattttcatctacttaaggaaatagggtattgtagcttaggctgatcatacccttcatttcaaccttaagctctcaacctgcatccatccgacttgagctattaagtactttagttttatcgagtataagttaacagaaaaagtaaattaagctttgcctttactattttgaatttatatacattctggaaaaacttagaaactgttgtatatttcattagattaaattatatgaaaatgtgattgtttatagcaaagcctgtgagttgcatacaccctaaggaaaactccttaagtgctccttgaagagagaagaaacaattctgggtctggtctttttaagaacaaagctagactactgtatgttagcactgtacattaatagtctgttgtgaagcttgagcagtttcctgcatagccttgatccttcaccgttggcattgaaaatagcagtatccctgatgtacttaaaacttaaagtcaggttttggtatatttatttgtaagtcttaatttcctctaaatactatatctctttagcgagacaacctgaaatttattagcacatttgggtatctcttgcttggcattatggccagtgttaactattcagtggtgaaaaaattacccctcaagacactggagtgaccccagatgtgtgtagtaagtggcatggttcaactgtgtggttaatgataaatatatgacttagtcggtatgatctggaaagacttgattgaaagataattcagctgacataaggatgagtgaggagtggcaaactggataaaagagtcaagagacctgtattccagtgactcctgttttgtttaagcattagcaagatctgtctggggaaactggatagggcagttttcttccatgtttagtttttgtctcaacatttggaagctattgaaggttttaaaatggtgtgtattgtttttttttggggggggggtggccagaatagtgggtcatctaataaaactgccatttaaaagatcaaaaaaaaaaaaaaaaaaaaaaaaa

SEQ ID NO: 20 - protein, 707 aa, Mus musculus
MPSATSHSGSGSKSSGPPPPSGSSGSEAAAGAAAPASQHPATGTGAVQTEAMKQILGVIDKKLRNLEKKKGKLDDYQERMNKGERLNQDQLDAVSKYQEVTNNLEFAKELQRSFMALSQDIQKTIKKTARREQLMREEAEQKRLKTVLELQYVLDKLGDDDVRTDLKQGLSGVPILSEEELSLLDEFYKLVDPERDMSLRLNEQYEHASIHLWDLLEGKEKPVCGTTYKALKEIVERVFQSNYFDSTHNHQNGLCEEEEAASAPTVEDQVAEAEPEPAEEYTEQSEVESTEYVNRQFMAETQFSSGEKEQVDEWTVETVEVVNSLQQQPQAASPSVPEPHSLTPVAQSDPLVRRQRVQDLMAQMQGPYNFIQDSMLDFENQTLDPAIVSAQPMNPTQNMDMPQLVCPQVHSESRLAQSNQVPVQPEATQVPLVSSTSEGYTASQPLYQPSHATEQRPQKEPMDQIQATISLNTDQTTASSSLPAASQPQVFQAGTSKPLHSSGINVNAAPFQSMQTVFNMNAPVPPANEPETLKQQSQYQATYNQSFSSQPHQVEQTELQQDQLQTVVGTYHGSQDQPHQVPGNHQQPPQQNTGFPRSSQPYYNSRGVSRGGSRGARGLMNGYRGPANGFRGGYDGYRPSFSNTPNSGYSQSQFTAPRDYSGYQRDGYQQNFKRGSGQSGPRGAPRGRGGPPRPNRGMPQMNTQQVN

SEQ ID NO: 21 - DNA, 6141 bp, Mus musculus
  CDS (139)..(2262)
cccaccgcgcgcgcgcgtagccgcctgcccgcccgcccgctgcgcgttttgtcccgcgtctctccccgtccgtctcctgacttgctggtcttgtccttccctcccgcttttttcctctcctctcttctcggtctaaagatgccctcggccaccagccacagcggaagcggcagcaaatcgtcgggaccgccgccgccgtccggttcctccgggagtgaggcggcggccggggcagctgcgccggcttctcagcatccggcaaccggcaccggcgccgtccagaccgaggccatgaagcagattctcggcgtaatcgacaagaaacttcggaacctggagaagaaaaagggtaaacttgatgattaccaggaacgaatgaataaaggggaaaggctcaatcaagaccagctggatgccgtatctaagtaccaggaagtcacaaataatttggagtttgcaaaggaattacagaggagtttcatggcattaagtcaagatattcagaaaacaataaagaagacagcacgtcgggaacagcttatgagagaagaagcagaacagaagcgcttaaaaactgtacttgagttacagtatgtattggataagctgggagatgatgatgtgagaacagatctgaaacaaggtttgagtggagtgccaatattgtctgaggaggagttgtcattgctggatgagttctacaagctcgtagatcctgagcgtgacatgagtttaaggttaaatgagcagtatgaacatgcctcaattcacttgtgggatttgctggaagggaaagaaaagcctgtgtgtggaacaacctataaagctctaaaggaaattgttgagcgtgttttccagtcaaactactttgatagcactcacaatcatcaaaatgggttgtgtgaggaggaagaggcggcttcagcgcccacagtggaggaccaggtagctgaagctgaacctgagccagcggaagaatacacagagcaaagtgaggttgaatcaacagagtatgtcaataggcagttcatggcagaaacacagttcagcagtggtgagaaggagcaagtggatgagtggacagttgaaacagttgaggttgtaaactcactccagcagcaacctcaggctgcgtccccttcagtcccagagccccactctttgactccagtggctcagtcagatccacttgtgagaaggcagcgtgtacaagatcttatggcacaaatgcaagggccctataatttcatacaggattcaatgttggattttgaaaatcagacgcttgatcctgccattgtatccgcacagcctatgaaccctacccagaacatggatatgcctcagctggtttgccctcaggttcattctgaatctagacttgcccaatctaatcaagttcctgtacaaccagaagccacacaggttcctttggtttcatccacaagtgaggggtatacagcatctcagcccttgtaccagccatctcatgctacggagcagcggccgcagaaagagccaatggatcagattcaggcaacaatatctttgaatacagaccagactacagcatcctcatcccttcctgctgcttctcagcctcaagtgttccaggctgggacaagtaaacctttgcacagcagtggaatcaatgtaaatgcagctccattccagtccatgcaaacggtgttcaatatgaatgctccagtccctcctgctaatgaaccagaaacgttaaaacaacagagtcagtaccaggccacttataaccagagtttttccagtcagcctcaccaagtggaacaaacagagcttcaacaagaccaactgcaaacggtggttggcacttaccatggatcccaggaccagcctcatcaagtgcctggtaaccaccagcaacccccacagcagaacactggctttccacgtagcagtcagccttattacaacagtcgtggggtatctcgaggagggtctcgtggtgccagaggcttgatgaatggatacaggggccctgccaatggatttagaggaggatatgatggttaccgcccttcattctcgaacactccaaacagtggttattcacagtctcagttcactgctccccgggactactctggttaccagcgggatggatatcagcagaatttcaagcgaggctctgggcagagtggaccacggggagccccacgaggtcgtggagggcccccaagacccaacagagggatgccgcaaatgaacactcagcaagtgaattaatgtgatacacaggattatgtttaatcgccaaaaacacactggccagtgtaccataatatgttaccagaagagttattatctatttgttctccctttcaggaaacttattgtaaagggactgttttcatcccataaagacaggactgcaattgtcagctttacattacctggatatggaaggaaactatttttattctgcatgttctgtcctaagcgtcatcttgagccttgcacacaatacaatactcagattcctcacccttgcttaggagtaaaacattatatacttatggggtgataatatctccatagttagttgaagtggcttggaaaaaaaatgcaagattgaatttttgaccttggataaaatctacaatcagccctagaactattcagtggtaattgacaaagttaaagcattttctttgaaaggaagatggaaggagtggagtgtggtttagcaaaactgcatttcatagctttcccattaaattggagcaccgacagattaaaagcataccaaattatgcatgggtccttactcacacaagtgaggctggctaccagccttgacatagcactcactagtcttctggccaaacgactgtgattaaaacacatgtaaattgctctttagtagtggatactgtgtaagacaaagccaaattgcaaatcaggctttgattggctcttctggaaaatatgcatcaaatatgggggataatctggatgggctgctgctgtgctcaatgtgaactatttagatacctttggaacacttaacagtttctctgaacaatgacttacatggggattggtcctgtttgtcattcctcaccataattgcattgtcatcactaatccttggatcttgctgtattgttactcaaattggtaataggtactgatggaaatcgctaatggatggataatcataacacttttggtcacatgttttctcctgcagcctgaaagttcttaaagaaaaagatatcaaatgcctgctgctaccacccttttaaattgctatctttagaaaagcaccggtatgtgttttagattcatttccctgttttagggaaatgacaggcagtagtttcagttctgatggcaaaacaaataaaaacatgtttctaaaagttgtatcttgaaacactggtgttcaacagctagcagctaaagtaattcaacccatgcattgctagtgtcacagcctttggttatgtctagtagctgtttctgaagtattttcatttatcttttgtcaaatttaaccctgtttgaattctctcctttcctcaaggagacacttatgttcaaagtgttgattctttgccttaggtgcatagagagtagacagtttggagatggaaaggttagcagtgacttagccatatgttctgtgttggaatttgtgctagcagtttgagcactagctctgcgtgcctatgaactgaatgctgcttgtcccattccattttatgtcatggagaaataattccacttggtaacacaaaggctaagttaatgttattttctgtacagaaattaaattttacttttagccttttgtaaactttttttttttttttccaagccggtatcagctactcaaaacaattctcagatattcatcattagacaactggagtttttgctggttttgtagcctactaaaactgctgaggctgttgaacattccacattcaaaagttttgtagggtggtggataatggggaagcttcaatgtttattttaaaataaataaaataagttcttgacttttctcatgtgtggttatggtacatcatattggaagggttatctgtttacttttgccaagactattttgccagcacctacacttgtgtgctttaaaagacaactacctgggatgtaccacaaccatatgttaattgtattttattgggatggataaaatgtttgtggtttattggataatccctagatggtgtgttacgtgtgtagaatataattttatgatagtaagaaagcaaaattgaagaaaataagtttagtattgaatttgagttctgaagtgaattcagggaatgtctcacgtttcgggcttctacccaaagtgtagggcagaaggtgtaaaagttgtttgtagtttgacttgtttattttttaagttgcttattcctttcaacagcaacatatcattagctgtcattctaccattgcagttctagtgagttttaacgtctgcattcaagactgttttaaaagcaacctcactggacagagaactgctaaagtcttttccttaagatctgagtctttgttactcagtatcttctataatatgcaaatgcttgtctagaggcagaagaccttttgtttggtcaagtgtgtattttaccagagtacagggaactgatggtcctacatgtctcttagtgtagtaagactataaaatcttttgtacatgcacaattcacagtatgtttagataccacgtgtataatgcccccccctcccccaggtagcatgccattgatgactttttgcttagggccattttattaccagggccttaatattcctaaaaagatgattttttttcatcctttctcctcttttgatcattgtatcttgatattaaaaacatgaccttccaatgattgtagtaaattaacttctatagttcttttgtctctatatgtattcatatatatgctattgtatagagacttcaaggagacatggagatgcatgcttattctcaggttcattcactaaggtgcttggcagacaaccagtttctaagtgcagaatgtagttaagcagcttcatatatgtgccaggcaatttgttttgttaaattttcatctacttaaggaaatagggtattgtagcttaggctgatcatacccttcatttcaaccttaagctctcaacctgcatccatccgacttgagctattaagtactttagttttatcgagtataagttaacagaaaaagtaaattaagctttgcctttactattttgaatttatatacattctggaaaaacttagaaactgttgtatatttcattagattaaattatatgaaaatgtgattgtttatagcaaagcctgtgagttgcatacaccctaaggaaaactccttaagtgctccttgaagagagaagaaacaattctgggtctggtctttttaagaacaaagctagactactgtatgttagcactgtacattaatagtctgttgtgaagcttgagcagtttcctgcatagccttgatccttcaccgttggcattgaaaatagcagtatccctgatgtacttaaaacttaaagtcaggttttggtatatttatttgtaagtcttaatttcctctaaatactatatctctttagcgagacaacctgaaatttattagcacatttgggtatctcttgcttggcattatggccagtgttaactattcagtggtgaaaaaattacccctcaagacactggagtgaccccagatgtgtgtagtaagtggcatggttcaactgtgtggttaatgataaatatatgacttagtcggtatgatctggaaagacttgattgaaagataattcagctgacataaggatgagtgaggagtggcaaactggataaaagagtcaagagacctgtattccagtgactcctgttttgtttaagcattagcaagatctgtctggggaaactggatagggcagttttcttccatgtttagtttttgtctcaacatttggaagctattgaaggttttaaaatggtgtgtattgtttttttttggggggggggtggccagaatagtgggtcatctaataaaactgccatttaaaagatcaaaaaaaaaaaaaaaaaaaaaaaaa

SEQ ID NO: 22 - protein, 707 aa, Mus musculus; identical to SEQ ID NO: 20

SEQ ID NO: 23 - DNA, 6114 bp, Mus musculus
  CDS (139)..(2235)
cccaccgcgcgcgcgcgtagccgcctgcccgcccgcccgctgcgcgttttgtcccgcgtctctccccgtccgtctcctgacttgctggtcttgtccttccctcccgcttttttcctctcctctcttctcggtctaaagatgccctcggccaccagccacagcggaagcggcagcaaatcgtcgggaccgccgccgccgtccggttcctccgggagtgaggcggcggccggggcagctgcgccggcttctcagcatccggcaaccggcaccggcgccgtccagaccgaggccatgaagcagattctcggcgtaatcgacaagaaacttcggaacctggagaagaaaaagggtaaacttgatgattaccaggaacgaatgaataaaggggaaaggctcaatcaagaccagctggatgccgtatctaagtaccaggaagtcacaaataatttggagtttgcaaaggaattacagaggagtttcatggcattaagtcaagatattcagaaaacaataaagaagacagcacgtcgggaacagcttatgagagaagaagcagaacagaagcgcttaaaaactgtacttgagttacagtatgtattggataagctgggagatgatgatgtgagaacagatctgaaacaaggtttgagtggagtgccaatattgtctgaggaggagttgtcattgctggatgagttctacaagctcgtagatcctgagcgtgacatgagtttaaggttaaatgagcagtatgaacatgcctcaattcacttgtgggatttgctggaagggaaagaaaagcctgtgtgtggaacaacctataaagctctaaaggaaattgttgagcgtgttttccagtcaaactactttgatagcactcacaatcatcaaaatgggttgtgtgaggaggaagaggcggcttcagcgcccacagtggaggaccaggtagctgaagctgaacctgagccagcggaagaatacacagagcaaagtgaggttgaatcaacagagtatgtcaataggcagttcatggcagaaacacagttcagcagtggtgagaaggagcaagtggatgagtggacagttgaaacagttgaggttgtaaactcactccagcagcaacctcaggctgcgtccccttcagtcccagagccccactctttgactccagtggctcagtcagatccacttgtgagaaggcagcgtgtacaagatcttatggcacaaatgcaagggccctataatttcatacagacgcttgatcctgccattgtatccgcacagcctatgaaccctacccagaacatggatatgcctcagctggtttgccctcaggttcattctgaatctagacttgcccaatctaatcaagttcctgtacaaccagaagccacacaggttcctttggtttcatccacaagtgaggggtatacagcatctcagcccttgtaccagccatctcatgctacggagcagcggccgcagaaagagccaatggatcagattcaggcaacaatatctttgaatacagaccagactacagcatcctcatcccttcctgctgcttctcagcctcaagtgttccaggctgggacaagtaaacctttgcacagcagtggaatcaatgtaaatgcagctccattccagtccatgcaaacggtgttcaatatgaatgctccagtccctcctgctaatgaaccagaaacgttaaaacaacagagtcagtaccaggccacttataaccagagtttttccagtcagcctcaccaagtggaacaaacagagcttcaacaagaccaactgcaaacggtggttggcacttaccatggatcccaggaccagcctcatcaagtgcctggtaaccaccagcaacccccacagcagaacactggctttccacgtagcagtcagccttattacaacagtcgtggggtatctcgaggagggtctcgtggtgccagaggcttgatgaatggatacaggggccctgccaatggatttagaggaggatatgatggttaccgcccttcattctcgaacactccaaacagtggttattcacagtctcagttcactgctccccgggactactctggttaccagcgggatggatatcagcagaatttcaagcgaggctctgggcagagtggaccacggggagccccacgaggtcgtggagggcccccaagacccaacagagggatgccgcaaatgaacactcagcaagtgaattaatgtgatacacaggattatgtttaatcgccaaaaacacactggccagtgtaccataatatgttaccagaagagttattatctatttgttctccctttcaggaaacttattgtaaagggactgttttcatcccataaagacaggactgcaattgtcagctttacattacctggatatggaaggaaactatttttattctgcatgttctgtcctaagcgtcatcttgagccttgcacacaatacaatactcagattcctcacccttgcttaggagtaaaacattatatacttatggggtgataatatctccatagttagttgaagtggcttggaaaaaaaatgcaagattgaatttttgaccttggataaaatctacaatcagccctagaactattcagtggtaattgacaaagttaaagcattttctttgaaaggaagatggaaggagtggagtgtggtttagcaaaactgcatttcatagctttcccattaaattggagcaccgacagattaaaagcataccaaattatgcatgggtccttactcacacaagtgaggctggctaccagccttgacatagcactcactagtcttctggccaaacgactgtgattaaaacacatgtaaattgctctttagtagtggatactgtgtaagacaaagccaaattgcaaatcaggctttgattggctcttctggaaaatatgcatcaaatatgggggataatctggatgggctgctgctgtgctcaatgtgaactatttagatacctttggaacacttaacagtttctctgaacaatgacttacatggggattggtcctgtttgtcattcctcaccataattgcattgtcatcactaatccttggatcttgctgtattgttactcaaattggtaataggtactgatggaaatcgctaatggatggataatcataacacttttggtcacatgttttctcctgcagcctgaaagttcttaaagaaaaagatatcaaatgcctgctgctaccacccttttaaattgctatctttagaaaagcaccggtatgtgttttagattcatttccctgttttagggaaatgacaggcagtagtttcagttctgatggcaaaacaaataaaaacatgtttctaaaagttgtatcttgaaacactggtgttcaacagctagcagctaaagtaattcaacccatgcattgctagtgtcacagcctttggttatgtctagtagctgtttctgaagtattttcatttatcttttgtcaaatttaaccctgtttgaattctctcctttcctcaaggagacacttatgttcaaagtgttgattctttgccttaggtgcatagagagtagacagtttggagatggaaaggttagcagtgacttagccatatgttctgtgttggaatttgtgctagcagtttgagcactagctctgcgtgcctatgaactgaatgctgcttgtcccattccattttatgtcatggagaaataattccacttggtaacacaaaggctaagttaatgttattttctgtacagaaattaaattttacttttagccttttgtaaactttttttttttttttccaagccggtatcagctactcaaaacaattctcagatattcatcattagacaactggagtttttgctggttttgtagcctactaaaactgctgaggctgttgaacattccacattcaaaagttttgtagggtggtggataatggggaagcttcaatgtttattttaaaataaataaaataagttcttgacttttctcatgtgtggttatggtacatcatattggaagggttatctgtttacttttgccaagactattttgccagcacctacacttgtgtgctttaaaagacaactacctgggatgtaccacaaccatatgttaattgtattttattgggatggataaaatgtttgtggtttattggataatccctagatggtgtgttacgtgtgtagaatataattttatgatagtaagaaagcaaaattgaagaaaataagtttagtattgaatttgagttctgaagtgaattcagggaatgtctcacgtttcgggcttctacccaaagtgtagggcagaaggtgtaaaagttgtttgtagtttgacttgtttattttttaagttgcttattcctttcaacagcaacatatcattagctgtcattctaccattgcagttctagtgagttttaacgtctgcattcaagactgttttaaaagcaacctcactggacagagaactgctaaagtcttttccttaagatctgagtctttgttactcagtatcttctataatatgcaaatgcttgtctagaggcagaagaccttttgtttggtcaagtgtgtattttaccagagtacagggaactgatggtcctacatgtctcttagtgtagtaagactataaaatcttttgtacatgcacaattcacagtatgtttagataccacgtgtataatgcccccccctcccccaggtagcatgccattgatgactttttgcttagggccattttattaccagggccttaatattcctaaaaagatgattttttttcatcctttctcctcttttgatcattgtatcttgatattaaaaacatgaccttccaatgattgtagtaaattaacttctatagttcttttgtctctatatgtattcatatatatgctattgtatagagacttcaaggagacatggagatgcatgcttattctcaggttcattcactaaggtgcttggcagacaaccagtttctaagtgcagaatgtagttaagcagcttcatatatgtgccaggcaatttgttttgttaaattttcatctacttaaggaaatagggtattgtagcttaggctgatcatacccttcatttcaaccttaagctctcaacctgcatccatccgacttgagctattaagtactttagttttatcgagtataagttaacagaaaaagtaaattaagctttgcctttactattttgaatttatatacattctggaaaaacttagaaactgttgtatatttcattagattaaattatatgaaaatgtgattgtttatagcaaagcctgtgagttgcatacaccctaaggaaaactccttaagtgctccttgaagagagaagaaacaattctgggtctggtctttttaagaacaaagctagactactgtatgttagcactgtacattaatagtctgttgtgaagcttgagcagtttcctgcatagccttgatccttcaccgttggcattgaaaatagcagtatccctgatgtacttaaaacttaaagtcaggttttggtatatttatttgtaagtcttaatttcctctaaatactatatctctttagcgagacaacctgaaatttattagcacatttgggtatctcttgcttggcattatggccagtgttaactattcagtggtgaaaaaattacccctcaagacactggagtgaccccagatgtgtgtagtaagtggcatggttcaactgtgtggttaatgataaatatatgacttagtcggtatgatctggaaagacttgattgaaagataattcagctgacataaggatgagtgaggagtggcaaactggataaaagagtcaagagacctgtattccagtgactcctgttttgtttaagcattagcaagatctgtctggggaaactggatagggcagttttcttccatgtttagtttttgtctcaacatttggaagctattgaaggttttaaaatggtgtgtattgtttttttttggggggggggtggccagaatagtgggtcatctaataaaactgccatttaaaagatcaaaaaaaaaaaaaaaaaaaaaaaaa

SEQ ID NO: 24 - protein, 698 aa, Mus musculus
MPSATSHSGSGSKSSGPPPPSGSSGSEAAAGAAAPASQHPATGTGAVQTEAMKQILGVIDKKLRNLEKKKGKLDDYQERMNKGERLNQDQLDAVSKYQEVTNNLEFAKELQRSFMALSQDIQKTIKKTARREQLMREEAEQKRLKTVLELQYVLDKLGDDDVRTDLKQGLSGVPILSEEELSLLDEFYKLVDPERDMSLRLNEQYEHASIHLWDLLEGKEKPVCGTTYKALKEIVERVFQSNYFDSTHNHQNGLCEEEEAASAPTVEDQVAEAEPEPAEEYTEQSEVESTEYVNRQFMAETQFSSGEKEQVDEWTVETVEVVNSLQQQPQAASPSVPEPHSLTPVAQSDPLVRRQRVQDLMAQMQGPYNFIQTLDPAIVSAQPMNPTQNMDMPQLVCPQVHSESRLAQSNQVPVQPEATQVPLVSSTSEGYTASQPLYQPSHATEQRPQKEPMDQIQATISLNTDQTTASSSLPAASQPQVFQAGTSKPLHSSGINVNAAPFQSMQTVFNMNAPVPPANEPETLKQQSQYQATYNQSFSSQPHQVEQTELQQDQLQTVVGTYHGSQDQPHQVPGNHQQPPQQNTGFPRSSQPYYNSRGVSRGGSRGARGLMNGYRGPANGFRGGYDGYRPSFSNTPNSGYSQSQFTAPRDYSGYQRDGYQQNFKRGSGQSGPRGAPRGRGGPPRPNRGMPQMNTQQVN

SEQ ID NO: 25 - DNA, 3548 bp, Mus musculus
  CDS (179)..(2257)
gctggctggctaagtccctcccgcgccggctcttgtcccactaggagcagctcagagccgcggggacagggcgaagcggcctgcgcccacggagcgcacgtctctgttctcaacgcagcaccacccttgcccccctcggctgcccactccagacgtccagcggctccgcgcgcgcacgatgccctcggccaccagccacagcggaagcggcagcaaatcgtcgggaccgccgccgccgtccggttcctccgggagtgaggcggcggccggggcagctgcgccggcttctcagcatccggcaaccggcaccggcgccgtccagaccgaggccatgaagcagattctcggcgtaatcgacaagaaacttcggaacctggagaagaaaaagggtaaacttgatgattaccaggaacgaatgaataaaggggaaaggctcaatcaagaccagctggatgccgtatctaagtaccaggaagtcacaaataatttggagtttgcaaaggaattacagaggagtttcatggcattaagtcaagatattcagaaaacaataaagaagacagcacgtcgggaacagcttatgagagaagaagcagaacagaagcgcttaaaaactgtacttgagttacagtatgtattggataagctgggagatgatgatgtgagaacagatctgaaacaaggtttgagtggagtgccaatattgtctgaggaggagttgtcattgctggatgagttctacaagctcgtagatcctgagcgtgacatgagtttaaggttaaatgagcagtatgaacatgcctcaattcacttgtgggatttgctggaagggaaagaaaagcctgtgtgtggaacaacctataaagctctaaaggaaattgttgagcgtgttttccagtcaaactactttgatagcactcacaatcatcaaaatgggttgtgtgaggaggaagaggcggcttcagcgcccacagtggaggaccaggtagctgaagctgaacctgagccagcggaagaatacacagagcaaagtgaggttgaatcaacagagtatgtcaataggcagttcatggcagaaacacagttcagcagtggtgagaaggagcaagtggatgagtggacagttgaaacagttgaggttgtaaactcactccagcagcaacctcaggctgcgtccccttcagtcccagagccccactctttgactccagtggctcagtcagatccacttgtgagaaggcagcgtgtacaagatcttatggcacaaatgcaagggccctataatttcatacaggattcaatgttggattttgaaaatcagacgcttgatcctgccattgtatccgcacagcctatgaaccctacccagaacatggatatgcctcagctggtttgccctcaggttcattctgaatctagacttgcccaatctaatcaagttcctgtacaaccagaagccacacaggttcctttggtttcatccacaagtgaggggtatacagcatctcagcccttgtaccagccatctcatgctacggagcagcggccgcagaaagagccaatggatcagattcaggcaacaatatctttgaatacagaccagactacagcatcctcatcccttcctgctgcttctcagcctcaagtgttccaggctgggacaagtaaacctttgcacagcagtggaatcaatgtaaatgcagctccattccagtccatgcaaacggtgttcaatatgaatgctccagtccctcctgctaatgaaccagaaacgttaaaacaacagagtcagtaccaggccacttataaccagagtttttccagtcagcctcaccaagtggaacaaacagagcttcaacaagaccaactgcaaacggtggttggcacttaccatggatcccaggaccagcctcatcaagtgcctggtaaccaccagcaacccccacagcagaacactggctttccacgtagcagtcagccttattacaacagtcgtggggtatctcgaggagggtctcgtggtgccagaggcttgatgaatggatacaggggccctgccaatggatttagaggaggatatgatggttaccgcccttcattctcgaacactccaaacagtggttattcacagtctcagttcactgctccccgggactactctggttaccagcgggatggatatcagcagaatttcaagcgaggctctgggcagagtggaccacggggagccccacgaggtaatatattgtggtggtgatcctagctcctatgtggagcttctgttctggccttggaagaactgttcatagtccgcatgtaggttacatgttaggaatacatttatcttttccagacttgttgctaaagattaaatgaaatgctctgtttctaaaatttcatcttgaatccaaattttaatttttgaatgactttccctgctgttgtcttcaaaatcagaacattttctctgcctcagaaaagcgtttttccaactggaaatttatttttcaggtcttaaaacctgctaaatgtttttaggaagtacctactgaaactttttgtaagacatttttggaacgagcttgaacatttatataaatttattaccctctttgatttttgaaacatgcatattatatttaggctgagaagcccttcaaatggccagataagccacagttttagctagagaaccatttagaattgacataactaatctaaacttgaacacttttaggaccaatgttagtgttctaaataccaacatatttctgatgtttaaacagatctcccaaattcttaggaccttgatgtcattaaaatttagaatgacaagcttaagaggctttagtttcatttgtttttcaagtaatgaaaaataatttcttacatgggcagatagttaatttgttgaacaattacaggtagcatttcatgtaatctgatgttctaaatggttctcttattgaaggaggttaaagaattaggtttcttacagtttttggctggccatgacatgtataaaatgtatattaaggaggaattataaagtactttaatttgaatgctagtggcaattgatcattaagaaagtactttaaagcaaaaggttaatgggtcatctgggaaaaatactgaagtatcaaaggtatttgcatgtgaatgtgggttatgttcttctatcccaccttgtagcatattctatgaaagttgagttaaatgatagctaaaatatctgtttcaacagcatgtaaaaagttattttaactgttacaagtcattatacaattttgaatgttctgtagtttctttttaacagtttaggtacaaaggtctgttttcattctggtgctttttattaattttgatagtatgatgtcacttcctattgaaatgtaagctagcgtgtaccttagaatgtgagctccatgagagcaggtaccttgtttgtcttcactgctgtatctattcccaacgcctcatgacagtgcctggcacatagtaggcactcaataaatacttgttgaatgaatgaaaaaaaaaaaaaa

SEQ ID NO: 26 - protein, 692 aa, Mus musculus
MPSATSHSGSGSKSSGPPPPSGSSGSEAAAGAAAPASQHPATGTGAVQTEAMKQILGVIDKKLRNLEKKKGKLDDYQERMNKGERLNQDQLDAVSKYQEVTNNLEFAKELQRSFMALSQDIQKTIKKTARREQLMREEAEQKRLKTVLELQYVLDKLGDDDVRTDLKQGLSGVPILSEEELSLLDEFYKLVDPERDMSLRLNEQYEHASIHLWDLLEGKEKPVCGTTYKALKEIVERVFQSNYFDSTHNHQNGLCEEEEAASAPTVEDQVAEAEPEPAEEYTEQSEVESTEYVNRQFMAETQFSSGEKEQVDEWTVETVEVVNSLQQQPQAASPSVPEPHSLTPVAQSDPLVRRQRVQDLMAQMQGPYNFIQDSMLDFENQTLDPAIVSAQPMNPTQNMDMPQLVCPQVHSESRLAQSNQVPVQPEATQVPLVSSTSEGYTASQPLYQPSHATEQRPQKEPMDQIQATISLNTDQTTASSSLPAASQPQVFQAGTSKPLHSSGINVNAAPFQSMQTVFNMNAPVPPANEPETLKQQSQYQATYNQSFSSQPHQVEQTELQQDQLQTVVGTYHGSQDQPHQVPGNHQQPPQQNTGFPRSSQPYYNSRGVSRGGSRGARGLMNGYRGPANGFRGGYDGYRPSFSNTPNSGYSQSQFTAPRDYSGYQRDGYQQNFKRGSGQSGPRGAPRGNILWW

SEQ ID NO: 27 - DNA, 3508 bp, Mus musculus
  CDS (139)..(2217)
cccaccgcgcgcgcgcgtagccgcctgcccgcccgcccgctgcgcgttttgtcccgcgtctctccccgtccgtctcctgacttgctggtcttgtccttccctcccgcttttttcctctcctctcttctcggtctaaagatgccctcggccaccagccacagcggaagcggcagcaaatcgtcgggaccgccgccgccgtccggttcctccgggagtgaggcggcggccggggcagctgcgccggcttctcagcatccggcaaccggcaccggcgccgtccagaccgaggccatgaagcagattctcggcgtaatcgacaagaaacttcggaacctggagaagaaaaagggtaaacttgatgattaccaggaacgaatgaataaaggggaaaggctcaatcaagaccagctggatgccgtatctaagtaccaggaagtcacaaataatttggagtttgcaaaggaattacagaggagtttcatggcattaagtcaagatattcagaaaacaataaagaagacagcacgtcgggaacagcttatgagagaagaagcagaacagaagcgcttaaaaactgtacttgagttacagtatgtattggataagctgggagatgatgatgtgagaacagatctgaaacaaggtttgagtggagtgccaatattgtctgaggaggagttgtcattgctggatgagttctacaagctcgtagatcctgagcgtgacatgagtttaaggttaaatgagcagtatgaacatgcctcaattcacttgtgggatttgctggaagggaaagaaaagcctgtgtgtggaacaacctataaagctctaaaggaaattgttgagcgtgttttccagtcaaactactttgatagcactcacaatcatcaaaatgggttgtgtgaggaggaagaggcggcttcagcgcccacagtggaggaccaggtagctgaagctgaacctgagccagcggaagaatacacagagcaaagtgaggttgaatcaacagagtatgtcaataggcagttcatggcagaaacacagttcagcagtggtgagaaggagcaagtggatgagtggacagttgaaacagttgaggttgtaaactcactccagcagcaacctcaggctgcgtccccttcagtcccagagccccactctttgactccagtggctcagtcagatccacttgtgagaaggcagcgtgtacaagatcttatggcacaaatgcaagggccctataatttcatacaggattcaatgttggattttgaaaatcagacgcttgatcctgccattgtatccgcacagcctatgaaccctacccagaacatggatatgcctcagctggtttgccctcaggttcattctgaatctagacttgcccaatctaatcaagttcctgtacaaccagaagccacacaggttcctttggtttcatccacaagtgaggggtatacagcatctcagcccttgtaccagccatctcatgctacggagcagcggccgcagaaagagccaatggatcagattcaggcaacaatatctttgaatacagaccagactacagcatcctcatcccttcctgctgcttctcagcctcaagtgttccaggctgggacaagtaaacctttgcacagcagtggaatcaatgtaaatgcagctccattccagtccatgcaaacggtgttcaatatgaatgctccagtccctcctgctaatgaaccagaaacgttaaaacaacagagtcagtaccaggccacttataaccagagtttttccagtcagcctcaccaagtggaacaaacagagcttcaacaagaccaactgcaaacggtggttggcacttaccatggatcccaggaccagcctcatcaagtgcctggtaaccaccagcaacccccacagcagaacactggctttccacgtagcagtcagccttattacaacagtcgtggggtatctcgaggagggtctcgtggtgccagaggcttgatgaatggatacaggggccctgccaatggatttagaggaggatatgatggttaccgcccttcattctcgaacactccaaacagtggttattcacagtctcagttcactgctccccgggactactctggttaccagcgggatggatatcagcagaatttcaagcgaggctctgggcagagtggaccacggggagccccacgaggtaatatattgtggtggtgatcctagctcctatgtggagcttctgttctggccttggaagaactgttcatagtccgcatgtaggttacatgttaggaatacatttatcttttccagacttgttgctaaagattaaatgaaatgctctgtttctaaaatttcatcttgaatccaaattttaatttttgaatgactttccctgctgttgtcttcaaaatcagaacattttctctgcctcagaaaagcgtttttccaactggaaatttatttttcaggtcttaaaacctgctaaatgtttttaggaagtacctactgaaactttttgtaagacatttttggaacgagcttgaacatttatataaatttattaccctctttgatttttgaaacatgcatattatatttaggctgagaagcccttcaaatggccagataagccacagttttagctagagaaccatttagaattgacataactaatctaaacttgaacacttttaggaccaatgttagtgttctaaataccaacatatttctgatgtttaaacagatctcccaaattcttaggaccttgatgtcattaaaatttagaatgacaagcttaagaggctttagtttcatttgtttttcaagtaatgaaaaataatttcttacatgggcagatagttaatttgttgaacaattacaggtagcatttcatgtaatctgatgttctaaatggttctcttattgaaggaggttaaagaattaggtttcttacagtttttggctggccatgacatgtataaaatgtatattaaggaggaattataaagtactttaatttgaatgctagtggcaattgatcattaagaaagtactttaaagcaaaaggttaatgggtcatctgggaaaaatactgaagtatcaaaggtatttgcatgtgaatgtgggttatgttcttctatcccaccttgtagcatattctatgaaagttgagttaaatgatagctaaaatatctgtttcaacagcatgtaaaaagttattttaactgttacaagtcattatacaattttgaatgttctgtagtttctttttaacagtttaggtacaaaggtctgttttcattctggtgctttttattaattttgatagtatgatgtcacttcctattgaaatgtaagctagcgtgtaccttagaatgtgagctccatgagagcaggtaccttgtttgtcttcactgctgtatctattcccaacgcctcatgacagtgcctggcacatagtaggcactcaataaatacttgttgaatgaatgaaaaaaaaaaaaaa

SEQ ID NO: 28 - protein, 692 aa, Mus musculus; identical to SEQ ID NO: 26

SEQ ID NO: 29 - DNA, 2109 bp, Gallus gallus
  CDS (1)..(2109)
atgccctcggctaccaacggcaccatggcgagcagcagcgggaaggcgggcccgggcggcaacgagcaggccccggcggcggcagcggcggccccgcaggcgtcgggcggcagcatcacctcggttcagaccgaggccatgaagcagatcttgggagtgatcgacaaaaagctccgcaacctcgagaagaaaaagagcaaacttgacgattaccaggaacgaatgaacaagggggaacgtctaaatcaagatcaactggatgcagtgtcaaaataccaggaagtgacaaataacctggaattcgctaaagaactgcagaggagctttatggcactgagccaagatatccagaaaacaataaaaaagacggctcgcagggagcagctgatgagagaagaggctgagcagaagcgtttaaagactgtgctagagctgcagttcattttggacaagttgggtgacgatgaagtgcgcagtgacttgaaacaaggatcaaatggagtaccggtactgacagaggaggaactgacaatgctggatgaattttacaagctagtttaccctgaaagggacatgaacatgaggttgaatgagcagtatgagcaagcatctgttcacctgtgggacttactggaagggaaggaaaaacccgtttgtggaacaacctataaagccctgaaggaggttgttgaacgtattcttcaaactagttactttgatagcacccataaccatcagaacgggttatgtgaggaagaagaggcagcacccacacctgcagtagaagacactgtagcagaagctgagcctgatccagcagaagaatttactgaacctactgaagttgaatcgactgagtatgtaaacagacaattcatggcagagactcagttcagcagtagtgagaaggaacaggtagatgagtggacagttgaaacggttgaggttgtaaattcactgcagcaacaaacacaagctacatctcctccagttcctgaacctcatacactcactactgtggctcaagcagatcctcttgttagaagacagagagtacaggaccttatggcccagatgcagggtccatataacttcatgcaggactctatgctggagtttgagaaccagacacttgatcctgccattgtatctgcacagcccatgaatccagcacagaatttggacatgccgcaaatggtctgccctccagttcatactgagtcaagacttgcccagcctaatcaagttcctgtgcaaccagaagctacgcaggttcccttggtttcatctacaagtgagggatatacagcctcccagcccatgtatcagccttctcataccacagagcaacggccacagaaggaatccattgaccagattcaggcttcaatgtcactgaatgcagaccagaccccgtcatcatcatcacttcccactgcatcccagccgcaagttttccaagctggatctagcaaacctttgcatagcagcggaatcaatgttaatgcagctccattccaatccatgcaaacagtattcaacatgaatgcacctgttcctcctgttaatgagccagaagcccttaagcaacaaaatcagtaccaggccagttacaaccagagtttctccaatcagccacaccaagtagaacaatcagatcttcagcaagaacagctccagacagtggttggtacttaccatggttctccggaccagacccatcaagtggcaggaaaccaccagcaacctccccagcagaatactggatttccacgcaacagtcagccttattacaacagtcggggagtgtctcgtggtggatcacgtgggactcgtggattgatgaatggttacaggggacctgcaaatggatttagaggaggatatgatggctaccgtccttcattttccaacactccgaacagtggttacacgcagccccaatttaatgctcctcgagattattcaaactaccagcgggatggatatcagcagaacttcaaacgtggttctggacaaagtgggcctcggggagctcctcgaggtcgtggagggcccccaagaccaaacagagggatgcctcaaatgaacgctcagcaagtgaattaa

SEQ ID NO: 30 - protein, 702 aa, Gallus gallus
MPSATNGTMASSSGKAGPGGNEQAPAAAAAAPQASGGSITSVQTEAMKQILGVIDKKLRNLEKKKSKLDDYQERMNKGERLNQDQLDAVSKYQEVTNNLEFAKELQRSFMALSQDIQKTIKKTARREQLMREEAEQKRLKTVLELQFILDKLGDDEVRSDLKQGSNGVPVLTEEELTMLDEFYKLVYPERDMNMRLNEQYEQASVHLWDLLEGKEKPVCGTTYKALKEVVERILQTSYFDSTHNHQNGLCEEEEAAPTPAVEDTVAEAEPDPAEEFTEPTEVESTEYVNRQFMAETQFSSSEKEQVDEWTVETVEVVNSLQQQTQATSPPVPEPHTLTTVAQADPLVRRQRVQDLMAQMQGPYNFMQDSMLEFENQTLDPAIVSAQPMNPAQNLDMPQMVCPPVHTESRLAQPNQVPVQPEATQVPLVSSTSEGYTASQPMYQPSHTTEQRPQKESIDQIQASMSLNADQTPSSSSLPTASQPQVFQAGSSKPLHSSGINVNAAPFQSMQTVFNMNAPVPPVNEPEALKQQNQYQASYNQSFSNQPHQVEQSDLQQEQLQTVVGTYHGSPDQTHQVAGNHQQPPQQNTGFPRNSQPYYNSRGVSRGGSRGTRGLMNGYRGPANGFRGGYDGYRPSFSNTPNSGYTQPQFNAPRDYSNYQRDGYQQNFKRGSGQSGPRGAPRGRGGPPRPNRGMPQMNAQQVN

SEQ ID NO: 31 - protein, 63 aa, Homo sapiens
EEYTEQSEVESTEYVNRQFMAETQFTSGEKEQVDEWTVETVEVVNSLQQQPQAASPSVPEPHS

SEQ ID NO: 32 - protein, 18 aa, Homo sapiens
VFNMNAPVPPVNEPETLK

SEQ ID NO: 33 - protein, 16 aa, Homo sapiens
ATQVPLVSSTSEGYTA

SEQ ID NO: 34 - protein, 25 aa, Homo sapiens
QILGVIDKKLRNLEKKKGKLDDYQE

SEQ ID NO: 35 - protein, 23 aa, Homo sapiens
PRGRGGPPRPNRGMPQMNTQQVN

SEQ ID NO: 36 - protein, 5 aa, Gallus gallus
SYQMN

SEQ ID NO: 37 - protein, 17 aa, Gallus gallus
AINKFGNSTGHGAAVKG

SEQ ID NO: 38 - protein, 19 aa, Gallus gallus
HAYGYCGSGTWCAAGEIDA

SEQ ID NO: 39 - protein, 128 aa, Gallus gallus
AVTLDESGGGLQMSRGGLSLVCKASGFDFSSYQMNWIRQAPGKGLEFVAAINKFGNSTGHGAAVKGRVTISRDNGQSTVRLQLNNLRAEDTAIYFCTKHAYGYCGSGTWCAAGEIDAWGHGTEVIVSS

SEQ ID NO: 40 - protein, 9 aa, Gallus gallus
SGGGSYSYG

SEQ ID NO: 41 - protein, 7 aa, Gallus gallus
NNKRPSD

SEQ ID NO: 42 - protein, 10 aa, Gallus gallus
SGDSTDTAVF

SEQ ID NO: 43 - protein, 108 aa, Gallus gallus
QAASTQPSSVSANPGETVEITCSGGGSYSYGWFQQKSPGSAPVTVIYYNNKRPSDIPSRFSGSKSGSTGTLTITGVQADDEAVYYCGSGDSTDTAVFGAGTTLTVLGQ

SEQ ID NO: 44 - protein, 5 aa, Rabbit
SHSLG

SEQ ID NO: 45 - protein, 16 aa, Rabbit
DIRSGGSAYYANWAKG

SEQ ID NO: 46 - protein, 13 aa, Rabbit
TNGPSDLTNRLDL

SEQ ID NO: 47 - protein, 121 aa, Homo sapiens
EQSLVESGGGLVQPGGSLRLSCAASGFSLSSHSLGWVRQAPGKGLEWIGDIRSGGSAYYANWAKGRFTISRDNSKNTLYLQMNSLRAEDTAVYYCTRTNGPSDLTNRLDLWGQGTLVTVSS

SEQ ID NO: 48 - protein, 13 aa, Rabbit
QASQSLYNNENLA

SEQ ID NO: 49 - protein, 7 aa, Rabbit
GASTLAS

SEQ ID NO: 50 - protein, 13 aa, Rabbit
LGEFSCGSADCFA

SEQ ID NO: 51 - protein, 112 aa, Homo sapiens
QVLTQSPSSLSASVGDRVTINCQASQSLYNNENLAWFQQKPGKVPKRLIYGASTLASGVSSRFSGSGSGTEFTLTISSLQCEDFAIYYCLGEFSCGSADCFAFGGGTKVEIK

SEQ ID NO: 52 - protein, 4 aa, Gallus gallus
FDMG

SEQ ID NO: 53 - protein, 17 aa, Gallus gallus
QINDAGSRTWYATAVKG

SEQ ID NO: 54 - protein, 12 aa, Gallus gallus
GSGYVGAGAIDA

SEQ ID NO: 55 - protein, 120 aa, Gallus gallus
AVTLDESGGGLQTPGGGLSLVCKASGFTFSSFDMGWVRQAPGKGLEFVAQINDAGSRTWYATAVKGRATISRDNGQTTVRLQLNNLRAEDTGTYYCTRGSGYVGAGAIDAWGHGTEVIVS

SEQ ID NO: 56 - protein, 8 aa, Gallus gallus
SGGSGYYG

SEQ ID NO: 57 - protein, 7 aa, Gallus gallus
NDKRPSD

SEQ ID NO: 58 - protein, 10 aa, Gallus gallus
RYDSTDSGIF

SEQ ID NO: 59 - protein, 105 aa, Gallus gallus
AALTQPSSVSANPGETVKITCSGGSGYYGWYQQQKSPGSAPVTVIYQNDKRPSDIPSRFSGSGSGSTNTLTITGVQAEDEAVYFCGRYDSTDSGIFGAGTTLTVL

SEQ ID NO: 60 - protein, 6 aa, Oryctolagus cuniculus
GSYYMS

SEQ ID NO: 61 - protein, 17 aa, Oryctolagus cuniculus
YIYIGDGVTAYANWAKG

SEQ ID NO: 62 - protein, 4 aa, Oryctolagus cuniculus
GNKL

SEQ ID NO: 63 - protein, 112 aa, Oryctolagus cuniculus
QSLEESGGDLVKPGASLTLTCTASGFSFSGSYYMSWVRQAPGKGLEWIAYIYIGDGVTAYANWAKGRFTISKASSTTVTLQMTSLTAADTATYFCARGNKLWGPGTLVTVSS

SEQ ID NO: 64 - protein, 11 aa, Oryctolagus cuniculus
QASQSISSYLA

SEQ ID NO: 65 - protein, 7 aa, Oryctolagus cuniculus
DASNLDS

SEQ ID NO: 66 - protein, 14 aa, Oryctolagus cuniculus
QCTAVSSATIYGNA

SEQ ID NO: 67 - protein, 112 aa, Oryctolagus cuniculus
DVVMTQTPASVEAAVGGTVTIKCQASQSISSYLAWYQQKPGQPPKRLIYDASNLDSGVPSRFKGSGSGTDFTITISDLECADAATYYCQCTAVSSATIYGNAFGGGTEVVVK

SEQ ID NO: 68 - protein, 127 aa, Gallus gallus
AVTLDESGGGLQTPGGALSLVCKASGFTFSGYDMLWVRQAPGKGLEWVAGIGSTGGGTDYGAAVKGRATISRDNGQSTVRLQLNNLRAEDTATYYCAKVAGGCNSGYCRDSPGSIDAWGHGTEVIVS

SEQ ID NO: 69 - protein, 107 aa, Gallus gallus
AVTQQPASVSANPGETVKITCSGGGSRNYYGWYQQKSPGSVPVTVIYYDDQRPSNIPSRFSGALSGSTSTLTITGVQADDEAVYFCGSADSNTYEGSFGAGTTLTVL

SEQ ID NO: 70 - protein, 148 aa, Mus musculus
MEWSGVFIFLLSGTAGVLSEVQLHQFGAELVKPGASVKISCKASGYTFTDYNMDWVKQSHGKSLEWIGDINPNYDSTSYNQKFKGKATLTVDKSSSTAYMELRSLTSEDTAVYYCARSRSYDYEGFAYWGQGTLVTVSAAKTTPPSVY

SEQ ID NO: 71 - protein, 105 aa, Mus musculus
GLFCSVERCHYQLQSSQNLLSIVNRYHYMSGNPPKLLVYPALLIYEASITKSCVPDRFTRSGSGTNFTLTINFVHADDLIFYYCQHNRGSFLPSSSVQVPRRRSN

SEQ ID NO: 72 - protein, 109 aa, Mus musculus
PRASLGVSETLLCTSGFTFTDYYMSWVRQPPGKALEWLGFIRNKANGYTTEYSASVKGRFTISRDNSQSILYLQMNTLRAEDSATYYCARANWAFDYWGQGTTVTVSSK

SEQ ID NO: 73 - protein, 94 aa, Mus musculus
SGDRVSLSCRASQSISNYLHWYQQKSHESPRLLIKYASQSISGIPSRFSGSGSGTDFTLSINSVETEDFGMYFCQQSNSWPYTFGGGTKLEIKQ

SEQ ID NO: 74 - protein, 118 aa, Mus musculus
AAELVRPGTSVKVSCKASGYAFTNYLIVWIKQRPGQGLEWIGVISPGSGGTNYNEKFKGKAILTADKSSSTAYMQLSSLTSDEFAVYFCAREKIYDDYYEGYFDVWGAGPRHLLASLS

SEQ ID NO: 75 - protein, 107 aa, Mus musculus
GTRCDIRLTQTTSSLSASLGDRVTISCSASLGIGNYLNWYQQKPDGTVKLLIYYTSNLHSGVPSRFSGSGSGTDYSLTISNLEPEDIATYYCQHYSKLPLTFGAGPS

SEQ ID NO: 76 - protein, 113 aa, Mus musculus
GAELVRSGASVKMSCKASGYSFTDYNMYWVKQTPGQGLEWIGYIYPGNGGTNYNQKFKGKATLTADTSSSTAYMQISSLTSEDSAVYFCARDYDDGGYAMDYWGQGTTVTVSS

SEQ ID NO: 77 - protein, 117 aa, Mus musculus
LLLWLTGARCDIQMTQSPASLSASVGETVTITCRASGNIHNYLTWYQQKQGKSPQLLVYNAKTLADGVPSRFSGSGSGTQYSLKINRLQPEDFGSYYCQHFWNIPWTFGGGTKLNSR

SEQ ID NO: 78 - protein, 114 aa, Mus musculus
DAELVKPGASVKISCKASGYTFTDHSIHWVQQKPEQGLEWIGYISPGNGNIKYNEKFKGKATLTADKSSSTAYMQLNSLTSEDSAVYFCKRSLGRGGPYYFDYWGQGTTVTVSS

SEQ ID NO: 79 - protein, 108 aa, Mus musculus
DIVLTQAAPSLPVTPGESVSISCRSSKSLLHSNGNTYLYWFLQRPGQSPQLLIYRMSNLASGVPDRFSGSGSGTAFTLRISRVEAEDVGVYYCMQHREYPVTFGSGPN

SEQ ID NO: 80 - protein, 111 aa, Mus musculus
QVQLQQSGAELMKPGASVKISCKATGYTFSSYWIEWVKQRPGHGLEWIGEILPGSGSTNYNEKFKGKATFTADTSSNTAYMQLSSLTSEDSAVYYCASYYWYFDVWAQDHV

SEQ ID NO: 81 - protein, 109 aa, Mus musculus
IVMTQAAFSNPVTLGTSASISCRSSKNLLHSNGITYLYWYLQRPGQSPQLLIYRVSNLASGVPNRFSGSESGTDFTLRISRVEAEDVGVYYCAQLLELPYTSEGTKRWE

SEQ ID NO: 82 - protein, 109 aa, Mus musculus
GGGLVKPGGSLKLSCAASGFAFSSYDMSWIRQTPEKRLEWVAYISSGAGSTYYPDTVKGRFTVSRDNAKNTLYLQMSSLKSEDTAMYYCARHFYRFDYWGQGTTVTVSS

SEQ ID NO: 83 - protein, 113 aa, Mus musculus
LLLCVSGAPGSIVMTQTPKFLLVSAGDRITITCKASQSVSNDVAWYQQKPGQSPKLLIYYASNRYTGVPDRFTGSGYGTDFTFTISTVQAEDLAVYFCQQDDRFPLTFGAGPS

SEQ ID NO: 84 - protein, 112 aa, Mus musculus
QIQLVQSGPELKKPGETVKISCKASGYTFTNYGMNWVKQAPGKGLKWMGWINTYTGEPTYADDFKGRFAFSLETSASTAYLQINNLKNEDTATYFCATGAWFAYWAKDSSRH

SEQ ID NO: 85 - protein, 107 aa, Mus musculus
GVEGDIVMTQSHKFMSTSVGDRVSITCKASQDVGTAVAWYQQKPGQSPKLLIYWASTRHTGVPDRFTGSGSGTDFTLTISNVQSEDLADYFCQQYSSYPLTFGAGPS

SEQ ID NO: 86 - protein, 118 aa, Mus musculus
GGGLVQPGGSMKVSCVASGFSFIDFWMNWVRQSPEKGLEWVAEIRLKSNNYATHYAESVKGRFTISRDDSKSSVYLQMNNLRPEDTGIYYCTSLFYYYDGTSGFAYWGQGTTVTVLLK

SEQ ID NO: 87 - protein, 109 aa, Mus musculus
DIVMTQSPSSLTVTAGEKVTMHCKSSQSLLNSGDQKNYLTWYQQKPGQPPKLLIYWASTRESGVPDRFTGSGSGTDFTLTISSVQAEDLAVYYCQNDYDYPLTFGAGPS

SEQ ID NO: 88 - protein, 148 aa, Mus musculus; identical to SEQ ID NO: 70

SEQ ID NO: 89 - protein, 139 aa, Mus musculus
MSVLTQVLGLLLLWLTGARCDIQMTQSPASLSASVGETVTITCRASGNIHNYLAWYQQKQGKSPQLLVYNAKTLADGVPSRFSGSGSGTQYSLKINSLQPEDFGSYYCQHFWSTLTFGAGTKLELKRADAAPTVSNPYD

SEQ ID NO: 90 - protein, 100 aa, Mus musculus
DILQASGYSFTGYTMNWVKQSHGKNLEWIGLINPYNGGTSYNQKFKGKATLTVDKSSSTAYMELLSLTSEDSAVYYCARWGVWSAMDYWGQGTTVTVSSK

SEQ ID NO: 91 - protein, 90 aa, Mus musculus
DRVSITCKASQNVRTAVAWYQQKPRQSPKALIYLASNRDTGLPDRFPGRGSGTDFTLNITNVQSEDLEDYFCLQHCNYPNEFRGCTKVPI

SEQ ID NO: 92 - protein, 116 aa, Mus musculus
LQESGAELARPGASVKLSCKASGYTFTSYWMQWVKQRPGQGLEWIGAIYPGDGDTRYTQKFKGKATLTADKSSSTAYMQLSSLASEDSAVYYCARGEYGNYFAYWGQGTTVTVSSN

SEQ ID NO: 93 - protein, 100 aa, Mus musculus
TSDASLGERVTITCKASQDINSYLSWFQQKPGKSPKTLIYRANRLVDGVPSRFSGSGSGQDYSLTISSLEYEDMGIYYCLQYDEFPLTFGGGTKLEIKQK

SEQ ID NO: 94 - protein, 108 aa, Mus musculus
AWLSQLSCTASGFNIKDTYMHWVKQRPEQGLEWIGRIDPANGNTKYDPKFQGKATITADTSSNTAYLQLSSLTSEDTAVYYCARPIHYYYGSSLAYWGQGTTVTVSSK

SEQ ID NO: 95 - protein, 104 aa, Mus musculus
EFHAVSLGQRATISCRASESVDSYGNSFMHWYQQKPGQPPKLLIYRASNLESGIPARFSGSGSRTDFTLTINPVEADDVATYYCQQSNEDPGRSEVVPSWRSNK

SEQ ID NO: 96 - protein, 109 aa, Mus musculus; identical to SEQ ID NO: 72

SEQ ID NO: 97 - protein, 94 aa, Mus musculus; identical to SEQ ID NO: 73

SEQ ID NO: 98 - protein, 111 aa, Mus musculus
PACLPGGSLRLSCATSGFTFTDYYMSWVRQPPGKALEWLGFIRNKANGYTTEYSASVKGRFTISRDNSQSILYLQMNTLRAEDSATYYCARAPLLYYAMDYWGQGTTVTVS

SEQ ID NO: 99 - protein, 102 aa, Mus musculus
RLPFYSLEQRATISYRASKNVSTSGYSYMHWNQQKPGQPPKLLIYLVSNLESGVPARFSGSGSGTDFTLNIHPVEEEDAATYYCQHIRELTRSELVPSWKSN

SEQ ID NO: 100 - protein, 101 aa, Mus musculus
VSCKASGYTFTSYWMHWVKQRPGQGLEWIGMIDPSNSETRLNQKFKDKATLNVDKSSNTAYMQLSSLTSEDSAVYYCARGLRHYWYFDVWGQGTTVTVSSK

SEQ ID NO: 101 - protein, 99 aa, Mus musculus
TILWREGPFSYRASKSVSTSGYSYMHWNQQKPGQPPRLLIYLVSNLESGVPARFSGSGSGTDFTLNIHPVEEEDAATYYCQHIRELTRSEEVPSWRSNK

SEQ ID NO: 102 - protein, 110 aa, Mus musculus
GGGLVKPGGSLKLSCAASGFTFSSYGMSWVRQTPEKRLEWVATISSGGSYTYYPDSVKGRFTISRDNAKNTLYLQMSSLRSEDTAMYYCASLASYYFDYWGQGTTLTVSS

SEQ ID NO: 103 - protein, 113 aa, Mus musculus
GARCDVQMIQSPSSLSASLGDIVTMTCQASQGTSINLNWFQQKPGKAPKLLIYGASSLEDGVPSRFSGSCFGTDFTLTISSLEDEDMATYFCLQHSYLPPLTFGAGTKLELKR

SEQ ID NO: 104 - protein, 111 aa, Mus musculus
GPGLVQPSQSLSITCTVSGFSLTTYDLHWVRQSPGKGLEWLGVIWSGGSTDYNAAFISRLSISKDNSKSQVFFKMNSLQANDTAIYYCARNYGYSAWFAYWGQGTLVTVSA

SEQ ID NO: 105 - protein, 118 aa, Mus musculus
PASSSDVLMTQTPLSLPVSLGDQASISCRSSQSIVHSNGNTYLEWYLQKPGQSPKLLIYKVSNRFSGVPDRFSGSGSGTDFTLKISRVEAEDLGVYYCFQGSHVPLTFGAGTKLELKR

SEQ ID NO: 106 - protein, 114 aa, Mus musculus
GFELKKPGETVKISCKASGYTFTAYSMHWVKQTPGKGLKWLGWINTETGEPTYTDDFKGRFTFSLETSARIAYLQINDLKNEDTATYFCARRIYYFGRGGFDYWGQGTTVTVSS

SEQ ID NO: 107 - protein, 118 aa, Mus musculus
PASSSDVLMTQTPLSLPVRLGDQSSISCRSSQSIVHSNGNTYLEWYLQKPGQSPKLLIYKVSNRFSGVPDRFSGSGSGTDFTLKISRVEPEDLGVYYCFQGSHVPYTSEGDQAEIKLA

SEQ ID NO: 108 - protein, 114 aa, Mus musculus
GGGLVQPGGSMRLSCVASGFTFSNSWFNWVRQSPEKGLEWVAEIRLTSDNYAIYYAESVKGRFTISRDDSKSSVYLQMNNLRAEDTGIYYCTRPETARATFAYWGQGTTVTVSS

SEQ ID NO: 109 - protein, 118 aa, Mus musculus
PASTSDVLMTQTPLSLPVSLGDQASISCRSSQSIVHSNGNTYLEWYLQKPGQSPKVLIYKVFNRFSGVPDRFSGSGSGTDFTLKISRVEAEDLGVYYCFQGSHVPRTFGGGTKLNQTG

SEQ ID NO: 110 - protein, 111 aa, Mus musculus
GPDLVKPGASVKISCKASGYSFTAYYMHWVKQSHGKSLEWIGRVNPNNGGTTYNQKFKGKAILTVDKSSSTAYMELRSLTFEDSAVYYCARRIYYGYFDYWGQGTTVTVSS

SEQ ID NO: 111 - protein, 104 aa, Mus musculus
AFFAVSLGQRATISCKASQSVDYDGDSYMNWYQQKPGQPPKLLIYVASNLESGVPARFSGSGSGTDFTLNIHPVEEEDAATYYCQQSNEDPYTFGGGTKLEIKQ

SEQ ID NO: 112 - protein, 106 aa, Mus musculus
GAELVKPGASVKLSCTASGLNIRDIYMHWVKQRPEQGLEWIGKIDPANGNTKYDPKFQGKATITADTSSNTAYVQLSSLTSEDTAVYYCAGTGDYWGQGTTVTVSS

SEQ ID NO: 113 - protein, 112 aa, Mus musculus
GTCGDIVMSQSPSSLAVSAGEKVTMSCKSSQSLLNSRTRKNYLAWVQHKPGQSPRLLIYWASTRESGVPDRFTGSGSGTDFTLTISSVQAEDLAVYYCRQSYNLVTFGAGPS

SEQ ID NO: 114 - protein, 112 aa, Mus musculus
GPELVKPGASVKMSCKASGYTFTSYVMHWVKQKPGQGLEWIGYINPYNDGTKYNEKFKGKATLTSDKSSSTAYMELSSLTSEDSAVYYCARRYYYGSSGGYFDVWAQDHVRT

SEQ ID NO: 115 - protein, 108 aa, Mus musculus
DVQITQSPSYLAASPGETITINCRASKSISKYLAWYQEKPGKTNKLLIYSGSTLQSGIPSRFSGSGSGTDFTLTISSLEPEDFAMYYCQQHNEYPYTFGGGTKLEIKR

SEQ ID NO: 116 - protein, 113 aa, Mus musculus
GPELVKPGASVKISCKASGYSFTGYFMNWVMQSHGKSLEWIGRINPYNGDTFYNQKFKGKATLTVDKSSSTAHMELRSLASEDSAVYYCARRIHYYYGSSYYAMDYWGQEPHH

SEQ ID NO: 117 - protein, 108 aa, Mus musculus
DVQITQSPSYLAASPGETITINCRASKSISKYLAWYQEKPGKTNKLLIYSGSTLQSGIPSRFSGSGSGTDFTLTISSLEPEDFAMYYCQQHNEYPWTFGGGTKLEIKR

SEQ ID NO: 118 - protein, 113 aa, Mus musculus
GAGLVKPGASVKLSCKASGYTFTEYIIHWVKQRSGQGLEWIGWFYPGSGSIKYNEKFKDKATLTADKSSSTVYMELSRLTSEDSAVYFCARHEVYYDYDKSMLWTTGVKNLIR

SEQ ID NO: 119 - protein, 108 aa, Mus musculus
SPSSLAVSVGEKVTMSCKSSQSLLYSSNQKNYLAWYQQKPGQSPKLLIYWASTRESGVPDRFTGSGSGTDFTLTISSVKAEDLAVYYCQQYYSYPYTFGGGTKLEIKR

SEQ ID NO: 120 - protein, 113 aa, Mus musculus
GAELVRPGTSVKVSCKASVYAFTNYLIEWVKQRPGQGLEWIGVINPKSGGTKYNEKFRGKATLTADKSSSTAYMQLSSLTSGDSAVYFCAITGTDYWGQGTTLTVSSAKTTPP

SEQ ID NO: 121 - protein, 113 aa, Mus musculus
QGTRCDIQMTQTTSSLSASLGDRVTISCSASQGINNYLNWYQQKPDGTVKLLIYYTSSLRSGVPSRFSGSGSGTDYSLTISNLEPEDVATYYCQQYSKLPRTFGGGTKLEIKR

SEQ ID NO: 122 - protein, 121 aa, Homo sapiens
EVQLVESGGGLVQPGGSLRLSCAASGFSLSSHSLGWVRQAPGKGLEWIGDIRSGGSAYYANWAKGRFTISRDNSKNTLYLQMNSLRAEDTAVYYCTRTNGPSDLTNRLDLWGQGTLVTVSS

SEQ ID NO: 123 - protein, 112 aa, Homo sapiens; identical to SEQ ID NO: 51

SEQ ID NO: 124 - protein, 121 aa, Homo sapiens
EVQLVESGGGLVQPGGSLRLSCAASGFSLSSHSLGWVRQAPGKGLEWIGDIRSGGSAYYANWAKGRFTISRDNSKNTLYLQMNSLRAEDTAVYFCTRTNGPSDLTNRLDLWGQGTLVTVSS

SEQ ID NO: 125 - protein, 112 aa, Homo sapiens; identical to SEQ ID NO: 51

SEQ ID NO: 126 - protein, 121 aa, Homo sapiens; identical to SEQ ID NO: 122

SEQ ID NO: 127 - protein, 113 aa, Homo sapiens
EQVLTQSPSSLSASVGDRVTINCQASQSLYNNENLAWFQQKPGKVPKRLIYGASTLASGVSSRFSGSGSGTEFTLTISNLQPEDFAIYYCLGEFSCGSADCFAFGGGTKVEIK

SEQ ID NO: 128 - protein, 121 aa, Homo sapiens; identical to SEQ ID NO: 124

SEQ ID NO: 129 - protein, 113 aa, Homo sapiens
EIVLTQSPSSLSASVGDRVTINCQASQSLYNNENLAWFQQKPGKVPKRLIYGASTLASGVSSRFSGSGSGTEFTLTISNLQPEDFATYYCLGEFSCGSADCFAFGGGTKVEIK

SEQ ID NO: 130 - protein, 121 aa, Homo sapiens; identical to SEQ ID NO: 122

SEQ ID NO: 131 - protein, 113 aa, Homo sapiens; identical to SEQ ID NO: 129

SEQ ID NO: 132 - protein, 121 aa, Homo sapiens; identical to SEQ ID NO: 124

SEQ ID NO: 133 - protein, 113 aa, Homo sapiens; identical to SEQ ID NO: 127

SEQ ID NO: 134 - protein, 5 aa, Gallus gallus
GYDML

SEQ ID NO: 135 - protein, 17 aa, Gallus gallus
GIGSTGGGTDYGAAVKG

SEQ ID NO: 136 - protein, 19 aa, Gallus gallus
VAGGCNSGYCRDSPGSIDA

SEQ ID NO: 137 - protein, 10 aa, Gallus gallus
SGGGSRNYYG

SEQ ID NO: 138 - protein, 7 aa, Gallus gallus
DDQRPSN

SEQ ID NO: 139 - protein, 11 aa, Gallus gallus
SADSNTYEGSF

SEQ ID NO: 140 - protein, 5 aa, Mus musculus
DYNMD

SEQ ID NO: 141 - protein, 17 aa, Mus musculus
DINPNYDSTSYNQKFKG

SEQ ID NO: 142 - protein, 11 aa, Mus musculus
SRSYDYEGFAY

SEQ ID NO: 143 - protein, 11 aa, Mus musculus
LSIVNRYHYMS

SEQ ID NO: 144 - protein, 6 aa, Mus musculus
EASITK

SEQ ID NO: 145 - protein, 9 aa, Mus musculus
QHNRGSFLP

SEQ ID NO: 146 - protein, 5 aa, Mus musculus
DYYMS

SEQ ID NO: 147 - protein, 17 aa, Mus musculus
RNKANGYTTEYSASVKG

SEQ ID NO: 148 - protein, 9 aa, Mus musculus
ARANWAFDY

SEQ ID NO: 149 - protein, 11 aa, Mus musculus
RASQSISNYLH

SEQ ID NO: 150 - protein, 7 aa, Mus musculus
YASQSIS

SEQ ID NO: 151 - protein, 7 aa, Mus musculus
YASQSIS

SEQ ID NO: 152 - protein, 5 aa, Mus musculus
NYLIV

SEQ ID NO: 153 - protein, 17 aa, Mus musculus
VISPGSGGTNYNEKFKG

SEQ ID NO: 154 - protein, 11 aa, Mus musculus
EKIYDDYYEGY

SEQ ID NO: 155 - protein, 15 aa, Mus musculus
TISCSASLGIGNYLN

SEQ ID NO: 156 - protein, 7 aa, Mus musculus
TSNLHSG

SEQ ID NO: 157 - protein, 9 aa, Mus musculus
HYSKLPLTF

SEQ ID NO: 158 - protein, 5 aa, Mus musculus
DYNMY

SEQ ID NO: 159 - protein, 17 aa, Mus musculus
YIYPGNGGTNYNQKFKG

SEQ ID NO: 160 - protein, 11 aa, Mus musculus
DYDDGGYAMDY

SEQ ID NO: 161 - protein, 15 aa, Mus musculus
SVGETVTITCRASGN

SEQ ID NO: 162 - protein, 7 aa, Mus musculus
NAKTLAD

SEQ ID NO: 163 - protein, 9 aa, Mus musculus
QHFWNIPWT

SEQ ID NO: 164 - protein, 5 aa, Mus musculus
DHSIH

SEQ ID NO: 165 - protein, 17 aa, Mus musculus
YISPGNGNIKYNEKFKG

SEQ ID NO: 166 - protein, 12 aa, Mus musculus
SLGRGGPYYFDY

SEQ ID NO: 167 - protein, 16 aa, Mus musculus
RSSKSLLHSNGNTYLY

SEQ ID NO: 168 - protein, 7 aa, Mus musculus
RMSNLAS

SEQ ID NO: 169 - protein, 9 aa, Mus musculus
MQHREYPVT

SEQ ID NO: 170 - protein, 5 aa, Mus musculus
SYWIE

SEQ ID NO: 171 - protein, 17 aa, Mus musculus
EILPGSGSTNYNEKFKG

SEQ ID NO: 172 - protein, 11 aa, Mus musculus
YYWYFDVWAQD

SEQ ID NO: 173 - protein, 15 aa, Mus musculus
SSKNLLHSNGITYLY

SEQ ID NO: 174 - protein, 7 aa, Mus musculus
RVSNLAS

SEQ ID NO: 175 - protein, 9 aa, Mus musculus
AQLLELPYT

SEQ ID NO: 176 - protein, 5 aa, Mus musculus
SYDMS

SEQ ID NO: 177 - protein, 17 aa, Mus musculus
YISSGAGSTYYPDTVKG

SEQ ID NO: 178 - protein, 11 aa, Mus musculus
HFYRFDYWGQG

SEQ ID NO: 179 - protein, 15 aa, Mus musculus
SAGDRITITCKASQS

SEQ ID NO: 180 - protein, 7 aa, Mus musculus
YASNRYT

SEQ ID NO: 181 - protein, 9 aa, Mus musculus
QQDDRFPLT

SEQ ID NO: 182 - protein, 5 aa, Mus musculus
NYGMN

SEQ ID NO: 183 - protein, 17 aa, Mus musculus
WINTYTGEPTYADDFKG

SEQ ID NO: 184 - protein, 11 aa, Mus musculus
GAWFAYWAKDS

SEQ ID NO: 185 - protein, 15 aa, Mus musculus
SITCKASQDVGTAVA

SEQ ID NO: 186 - protein, 7 aa, Mus musculus
WASTRHT

SEQ ID NO: 187 - protein, 9 aa, Mus musculus
QQYSSYPLT

SEQ ID NO: 188 - protein, 5 aa, Mus musculus
DFWMN

SEQ ID NO: 189 - protein, 19 aa, Mus musculus
EIRLKSNNYATHYAESVKG

SEQ ID NO: 190 - protein, 13 aa, Mus musculus
LFYYYDGTSGFAY

SEQ ID NO: 191 - protein, 17 aa, Mus musculus
KSSQSLLNSGDQKNYLT

SEQ ID NO: 192 - protein, 7 aa, Mus musculus
WASTRES

SEQ ID NO: 193 - protein, 9 aa, Mus musculus
QNDYDYPLT

SEQ ID NO: 194 - protein, 5 aa, Mus musculus
DYNMD

SEQ ID NO: 195 - protein, 17 aa, Mus musculus
DINPNYDSTSYNQKFKG

SEQ ID NO: 196 - protein, 11 aa, Mus musculus
SRSYDYEGFAY

SEQ ID NO: 197 - protein, 11 aa, Mus musculus
RASGNIHNYLA

SEQ ID NO: 198 - protein, 7 aa, Mus musculus
NAKTLAD

SEQ ID NO: 199 - protein, 8 aa, Mus musculus
QHFWSTLT

SEQ ID NO: 200 - protein, 5 aa, Mus musculus
GYTMN

SEQ ID NO: 201 - protein, 16 aa, Mus musculus
NPYNGGTSYNQKFKGK

SEQ ID NO: 202 - protein, 9 aa, Mus musculus
WGVWSAMDY

SEQ ID NO: 203 - protein, 11 aa, Mus musculus
KASQNVRTAVA

SEQ ID NO: 204 - protein, 7 aa, Mus musculus
LASNRDT

SEQ ID NO: 205 - protein, 9 aa, Mus musculus
LQHCNYPNE

SEQ ID NO: 206 - protein, 5 aa, Mus musculus
SYWMQ

SEQ ID NO: 207 - protein, 17 aa, Mus musculus
AIYPGDGDTRYTQKFKG

SEQ ID NO: 208 - protein, 11 aa, Mus musculus
ARGEYGNYFAY

SEQ ID NO: 209 - protein, 11 aa, Mus musculus
KASQDINSYLS

SEQ ID NO: 210 - protein, 7 aa, Mus musculus
RANRLVD

SEQ ID NO: 211 - protein, 9 aa, Mus musculus
LQYDEFPLT

SEQ ID NO: 212 - protein, 5 aa, Mus musculus
DTYMH

SEQ ID NO: 213 - protein, 17 aa, Mus musculus
RIDPANGNTKYDPKFQG

SEQ ID NO: 214 - protein, 14 aa, Mus musculus
ARPIHYYYGSSLAY

SEQ ID NO: 215 - protein, 11 aa, Mus musculus
SVDSYGNSFMH

SEQ ID NO: 216 - protein, 7 aa, Mus musculus
RASNLES

SEQ ID NO: 217 - protein, 9 aa, Mus musculus
QQSNEDPGR

SEQ ID NO: 218 - protein, 5 aa, Mus musculus
DYYMS

SEQ ID NO: 219 - protein, 17 aa, Mus musculus
RNKANGYTTEYSASVKG

SEQ ID NO: 220 - protein, 9 aa, Mus musculus
ARANWAFDY

SEQ ID NO: 221 - protein, 11 aa, Mus musculus
RASQSISNYLH

SEQ ID NO: 222 - protein, 7 aa, Mus musculus
YASQSIS

SEQ ID NO: 223 - protein, 9 aa, Mus musculus
QQSNSWPYT

SEQ ID NO: 224 - protein, 5 aa, Mus musculus
DYYMS

SEQ ID NO: 225 - protein, 17 aa, Mus musculus
RNKANGYTTEYSASVKG

SEQ ID NO: 226 - protein, 12 aa, Mus musculus
ARAPLLYYAMDY

SEQ ID NO: 227 - protein, 11 aa, Mus musculus
NVSTSGYSYMH

SEQ ID NO: 228 - protein, 7 aa, Mus musculus
LVSNLES

SEQ ID NO: 229 - protein, 8 aa, Mus musculus
QHIRELTR

SEQ ID NO: 230 - protein, 5 aa, Mus musculus
SYWMH

SEQ ID NO: 231 - protein, 17 aa, Mus musculus
MIDPSNSETRLNQKFKD

SEQ ID NO: 232 - protein, 12 aa, Mus musculus
ARGLRHYWYFDV

SEQ ID NO: 233 - protein, 11 aa, Mus musculus
SVSTSGYSYMH

SEQ ID NO: 234 - protein, 7 aa, Mus musculus
LVSNLES

SEQ ID NO: 235 - protein, 9 aa, Mus musculus
QHIRELTRS

SEQ ID NO: 236 - protein, 5 aa, Mus musculus
SYGMS

SEQ ID NO: 237 - protein, 14 aa, Mus musculus
WVRQTPEKRLEWVA

SEQ ID NO: 238 - protein, 11 aa, Mus musculus
LASYYFDYWGQ

SEQ ID NO: 239 - protein, 15 aa, Mus musculus
TMTCQASQGTSINLN

SEQ ID NO: 240 - protein, 7 aa, Mus musculus
GASSLED

SEQ ID NO: 241 - protein, 11 aa, Mus musculus
LQHSYLPPLTF

SEQ ID NO: 242 - protein, 5 aa, Mus musculus
TYDLH

SEQ ID NO: 243 - protein, 16 aa, Mus musculus
VIWSGGSTDYNAAFIS

SEQ ID NO: 244 - protein, 11 aa, Mus musculus
NYGYSAWFAYW

SEQ ID NO: 245 - protein, 15 aa, Mus musculus
ASISCRSSQSIVHSN

SEQ ID NO: 246 - protein, 7 aa, Mus musculus
KVSNRFS

SEQ ID NO: 247 - protein, 9 aa, Mus musculus
FQGSHVPLT

SEQ ID NO: 248 - protein, 5 aa, Mus musculus
AYSMH

SEQ ID NO: 249 - protein, 17 aa, Mus musculus
WINTETGEPTYTDDFKG

SEQ ID NO: 250 - protein, 11 aa, Mus musculus
RIYYFGRGGFD

SEQ ID NO: 251 - protein, 15 aa, Mus musculus
SSISCRSSQSIVHSN

SEQ ID NO: 252 - protein, 7 aa, Mus musculus
KVSNRFS

SEQ ID NO: 253 - protein, 9 aa, Mus musculus
FQGSHVPYT

SEQ ID NO: 254 - protein, 5 aa, Mus musculus
NSWFN

SEQ ID NO: 255 - protein, 19 aa, Mus musculus
EIRLTSDNYAIYYAESVKG

SEQ ID NO: 256 - protein, 11 aa, Mus musculus
PETARATFAYW

SEQ ID NO: 257 - protein, 15 aa, Mus musculus
ASISCRSSQSIVHSN

SEQ ID NO: 258 - protein, 7 aa, Mus musculus
KVFNRFS

SEQ ID NO: 259 - protein, 9 aa, Mus musculus
FQGSHVPRT

SEQ ID NO: 260 - protein, 5 aa, Mus musculus
AYYMH

SEQ ID NO: 261 - protein, 17 aa, Mus musculus
RVNPNNGGTTYNQKFKG

SEQ ID NO: 262 - protein, 11 aa, Mus musculus
RIYYGYFDYWG

SEQ ID NO: 263 - protein, 15 aa, Mus musculus
KASQSVDYDGDSYMN

SEQ ID NO: 264 - protein, 7 aa, Mus musculus
VASNLES

SEQ ID NO: 265 - protein, 9 aa, Mus musculus
QQSNEDPYT

SEQ ID NO: 266 - protein, 4 aa, Mus musculus
DIYM

SEQ ID NO: 267 - protein, 17 aa, Mus musculus
KIDPANGNTKYDPKFQG

SEQ ID NO: 268 - protein, 11 aa, Mus musculus
TGDYWGQGTTV

SEQ ID NO: 269 - protein, 15 aa, Mus musculus
TMSCKSSQSLLNSRT

SEQ ID NO: 270 - protein, 7 aa, Mus musculus
WASTRES

SEQ ID NO: 271 - protein, 9 aa, Mus musculus
RQSYNLVTF

SEQ ID NO: 272 - protein, 5 aa, Mus musculus
SYVMH

SEQ ID NO: 273 - protein, 17 aa, Mus musculus
YINPYNDGTKYNEKFKG

SEQ ID NO: 274 - protein, 11 aa, Mus musculus
RYYYGSSGGYF

SEQ ID NO: 275 - protein, 15 aa, Mus musculus
RASKSISKYLAWYQE

SEQ ID NO: 276 - protein, 7 aa, Mus musculus
SGSTLQS

SEQ ID NO: 277 - protein, 9 aa, Mus musculus
QQHNEYPYT

SEQ ID NO: 278 - protein, 5 aa, Mus musculus
GYFMN

SEQ ID NO: 279 - protein, 17 aa, Mus musculus
RINPYNGDTFYNQKFKG

SEQ ID NO: 280 - protein, 11 aa, Mus musculus
RIHYYYGSSYY

SEQ ID NO: 281 - protein, 15 aa, Mus musculus
RASKSISKYLAWYQE

SEQ ID NO: 282 - protein, 7 aa, Mus musculus
SGSTLQS

SEQ ID NO: 283 - protein, 9 aa, Mus musculus
QQHNEYPWT

SEQ ID NO: 284 - protein, 5 aa, Mus musculus
EYIIH

SEQ ID NO: 285 - protein, 17 aa, Mus musculus
WFYPGSGSIKYNEKFKD

SEQ ID NO: 286 - protein, 11 aa, Mus musculus
HEVYYDYDKSM

SEQ ID NO: 287 - protein, 15 aa, Mus musculus
LYSSNQKNYLAWYQQ

SEQ ID NO: 288 - protein, 7 aa, Mus musculus
WASTRES

SEQ ID NO: 289 - protein, 9 aa, Mus musculus
QQYYSYPYT

SEQ ID NO: 290 - protein, 5 aa, Mus musculus
NYLIE

SEQ ID NO: 291 - protein, 19 aa, Mus musculus
VINPKSGGTKYNEKFRGKA

SEQ ID NO: 292 - protein, 11 aa, Mus musculus
TGTDYWGQGTT

SEQ ID NO: 293 - protein, 10 aa, Mus musculus
VTISCSASQG

SEQ ID NO: 294 - protein, 7 aa, Mus musculus
YTSSLRS

SEQ ID NO: 295 - protein, 9 aa, Mus musculus
QQYSKLPRT

SEQ ID NO: 296 - protein, 12 aa, Homo sapiens
FTSGEKEQVDEW

SEQ ID NO: 297 - protein, 16 aa, Homo sapiens
AEQKRLKTVLELQYVL

SEQ ID NO: 298 - protein, 16 aa, Homo sapiens
VERVFQSNYFDSTHNH

SEQ ID NO: 299 - protein, 16 aa, Homo sapiens
FQSMQTVFNMNAPVPP

SEQ ID NO: 300 - protein, 5 aa, Mus musculus
TNAMN

SEQ ID NO: 301 - protein, 17 aa, Mus musculus
RIRSKSNNYATYYADSV

SEQ ID NO: 302 - protein, 11 aa, Mus musculus
DWDGFLYFDYW

SEQ ID NO: 303 - protein, 112 aa, Mus musculus
GGGLVQPKGSLKLSCAASGFTFNTNAMNWVRQAPGKGLEWVARIRSKSNNYATYYADSVKDRFTISRDDSQSMLYLQMNNLKTEDTAMYYCVRDWDGFLYFDYWAKHHLTLF

SEQ ID NO: 304 - protein, 15 aa, Mus musculus
SVSTSGYSYMHWNQQ

SEQ ID NO: 305 - protein, 7 aa, Mus musculus
LVSNLES

SEQ ID NO: 306 - protein, 9 aa, Mus musculus
QHIRELTRS

SEQ ID NO: 307 - protein, 104 aa, Mus musculus
TQSPASLAVSLGQRATISYRASKSVSTSGYSYMHWNQQKPGQPPRLLIYLVSNLESGVPARFSGSGSGTDFTLNIHPVEEEDAATYYCQHIRELTRSEGGPSWK

SEQ ID NO: 308 - protein, 14 aa, Homo sapiens
PPVNEPETLKQQNQ

SEQ ID NO: 309 - protein, 12 aa, Homo sapiens
ETLKQQNQYQAS